European Patent Specification EP 4 032 985 B1, published March 13, 2024. Title: MICROPEPTIDES ET LEUR UTILISATION POUR MODULER L'EXPRESSION DE GENES. Applicant: CENTRE NATIONAL DE LA RECHERCHE SCIENTIFIQUE - CNRS UNIVERSITE PAUL SABATIER. The sequence listing filed with the application follows.

SEQUENCE LISTING (495 sequences)

SEQ ID NO: 1 - protein, 33 aa, Arabidopsis thaliana
MFCSIQCVARHLFPLHVREIKKATRAIKKGKTL

SEQ ID NO: 2 - protein, 24 aa, Arabidopsis thaliana
MRRQTSVPFACKRDKESDKSHKER

SEQ ID NO: 3 - protein, 37 aa, Arabidopsis thaliana
MVMFFLDLDKNPRFDLLKGLKWNLFSSHISPSLPPSL

SEQ ID NO: 4 - protein, 11 aa, Arabidopsis thaliana
MKDNFPLLLRL

SEQ ID NO: 5 - protein, 4 aa, Arabidopsis thaliana
MSDD

SEQ ID NO: 6 - protein, 16 aa, Arabidopsis thaliana
MIYINKYGSISAVEDD

SEQ ID NO: 7 - protein, 4 aa, Arabidopsis thaliana
MSQR

SEQ ID NO: 8 - protein, 16 aa, Arabidopsis lyrata
MTCPLLSLSFLLSKYI

SEQ ID NO: 9 - protein, 16 aa, Arabidopsis thaliana
MTWPLLSLSFLLSKYV

SEQ ID NO: 10 - protein, 18 aa, Capsella rubella
MTCTLSALSLSLNMFRVN

SEQ ID NO: 11 - protein, 5 aa, Arabidopsis thaliana
MFYLS

SEQ ID NO: 12 - protein, 37 aa, Arabidopsis thaliana
MVNTSSFFISSFILPLVLSESNCLLFRTIYKFSMVLY

SEQ ID NO: 13 - protein, 24 aa, Arabidopsis thaliana
MFCLLIPIFSFVFSPNRHLRLQEQ

SEQ ID NO: 14 - protein, 5 aa, Arabidopsis thaliana
MFSPQ

SEQ ID NO: 15 - protein, 23 aa, Arabidopsis thaliana
MKYIHILILFKSRSTYKLSTNHI

SEQ ID NO: 16 - protein, 10 aa, Arabidopsis thaliana
MKIPLFLPKL

SEQ ID NO: 17 - protein, 27 aa, Arabidopsis thaliana
MVSGQEDSWLKLSSLCFLFLSLLDSLI

SEQ ID NO: 18 - protein, 34 aa, Arabidopsis thaliana
MFLLIFLRLIMICVCSSTDFLRSVNYFCLFIYDL

SEQ ID NO: 19 - protein, 9 aa, Arabidopsis thaliana
MSTTQEHRS

SEQ ID NO: 20 - protein, 25 aa, Arabidopsis thaliana
MILKCWSSRFLRVSPYQNAHSLSLG

SEQ ID NO: 21 - protein, 13 aa, Arabidopsis lyrata
MPLAVIRQGIVWP

SEQ ID NO: 22 - protein, 24 aa, Arabidopsis lyrata
MPSWHDMVLLPYVKHTHANTRHIT

SEQ ID NO: 23 - protein, 8 aa, Arabidopsis lyrata
MTWFFCLT

SEQ ID NO: 24 - protein, 37 aa, Arabidopsis thaliana
MPSWHGMVLLPYVKHTHASTHTHTHNIYGCACELVFH

SEQ ID NO: 25 - protein, 22 aa, Arabidopsis thaliana
MAWYGSFALRKTHSRQHTHTHT

SEQ ID NO: 26 - protein, 8 aa, Arabidopsis thaliana
MVWFFCLT

SEQ ID NO: 27 - protein, 7 aa, Brassica rapa
MMIILWK

SEQ ID NO: 28 - protein, 24 aa, Brassica rapa
MLWAKLVSFSTLHSLVFLLSPSFA

SEQ ID NO: 29 - protein, 29 aa, Brassica rapa
MPSWHGIVILPFVKHTHANIHYSYSCVCI

SEQ ID NO: 30 - protein, 34 aa, Carica papaya
MIACHPYLPFPLFLSLTFYSIFFSPSPPSPSLPL

SEQ ID NO: 31 - protein, 53 aa, Carica papaya
MPSLLAFSPFPFSNILLNLLLPLPPFPLSAIITIIKPLSLSLPLSLSLSGFSV

SEQ ID NO: 32 - protein, 15 aa, Capsella rubella
MELKGLRTWQLLDKV

SEQ ID NO: 33 - protein, 14 aa, Capsella rubella
MPSWHGMACFYCLT

SEQ ID NO: 34 - protein, 24 aa, Capsella rubella
MAWHGMFLLPYVKHTHANTYSLYM

SEQ ID NO: 35 - protein, 35 aa, Gossypium raimondii
MMRSRILKFQYRFGMGIGGRKQLKNQLCQIQGRIS

SEQ ID NO: 36 - protein, 10 aa, Gossypium raimondii
MSNSRSYQLK

SEQ ID NO: 37 - protein, 17 aa, Gossypium raimondii
MNEDLEISTRKRTPQLC

SEQ ID NO: 38 - protein, 12 aa, Medicago truncatula
MPKFDIFFYIFV

SEQ ID NO: 39 - protein, 83 aa, Medicago truncatula
MSYISLSPKLLPINTKPFPWLVQFNFYFSSNTKCNKLHFLGEKLLVGEAGHVQILFLIHSLIMHINIFCTCSPSPTRLPHPSL

SEQ ID NO: 40 - protein, 20 aa, Oryza sativa
MQTHSNTPQSTYSLSLSLSE

SEQ ID NO: 41 - protein, 15 aa, Oryza sativa
MCVCDINMHSMLMLL

SEQ ID NO: 42 - protein, 25 aa, Arabidopsis lyrata
MRIKLFQLRGMLSGSRILYIYTCVC

SEQ ID NO: 43 - protein, 18 aa, Arabidopsis thaliana
MRVKLFQLRGMLSGSRIL

SEQ ID NO: 44 - protein, 36 aa, Brassica carinata
MRMKLFQLRGMLSGSRILYIHKYVYMLIQVFDHICI

SEQ ID NO: 45 - protein, 27 aa, Brassica juncea
MRMKLFQLRGMLSGSRILYIHKYVYIC

SEQ ID NO: 46 - protein, 36 aa, Brassica napus
MRMKLFQLRGMLSGSRILYIHKYVYMIIQVFDHICI

SEQ ID NO: 47 - protein, 36 aa, Brassica oleracea; identical to SEQ ID NO: 44

SEQ ID NO: 48 - protein, 27 aa, Brassica rapa
MRMKLFQLRGMLSGSRILYIHKYVYIC

SEQ ID NO: 49 - protein, 19 aa, Arabidopsis thaliana
MLDLFRSNNRIEPSDFRFD

SEQ ID NO: 50 - protein, 4 aa, Arabidopsis thaliana
MRDR

SEQ ID NO: 51 - protein, 10 aa, Arabidopsis thaliana
MNRKISLSLS

SEQ ID NO: 52 - protein, 8 aa, Arabidopsis thaliana
MMGCFVGF

SEQ ID NO: 53 - protein, 8 aa, Arabidopsis thaliana
MQEETYEG

SEQ ID NO: 54 - protein, 59 aa, Arabidopsis thaliana
MPHTNLKDLFIFSPNVFFSFAIYLHNSWNKNYIHKRENFHNTSFALIFFFSSIMSINYG

SEQ ID NO: 55 - protein, 39 aa, Arabidopsis thaliana
MFFFRLLFISTILGTKTTFTNERIFTTPLLLSFFFFRPL

SEQ ID NO: 56 - protein, 6 aa, Arabidopsis thaliana
MRHKES

SEQ ID NO: 57 - protein, 34 aa, Arabidopsis thaliana
MNLLKKERQRRRQRSIGSHCIASLVLKDGYMKKI

SEQ ID NO: 58 - protein, 9 aa, Arabidopsis thaliana
MVLSGKLTF

SEQ ID NO: 59 - protein, 20 aa, Medicago truncatula
MLLHRLSKFCKIERDIVYIS

SEQ ID NO: 60 - protein, 5 aa, Medicago truncatula
MKIEE

SEQ ID NO: 61 - protein, 34 aa, Zea mays
MHLPSTPSRPPPQHTSLSFLGKEMTKGTTTACFG

SEQ ID NO: 62 - protein, 10 aa, Arabidopsis thaliana
MLSLSHFHIC

SEQ ID NO: 63 - protein, 23 aa, Medicago truncatula
MMVFGKPKKAMLVRFNPKTDLHV

SEQ ID NO: 64 - protein, 10 aa, Medicago truncatula
MASAAKVYMA

SEQ ID NO: 65 - protein, 6 aa, Arabidopsis thaliana
MASKIW

SEQ ID NO: 66 - protein, 10 aa, Arabidopsis thaliana
MVRFQLSIRD

SEQ ID NO: 67 - protein, 12 aa, Arabidopsis thaliana
MCTYYYLINKYF

SEQ ID NO: 68 - protein, 11 aa, Arabidopsis thaliana
MFPAKWCRLES

SEQ ID NO: 69 - protein, 22 aa, Arabidopsis thaliana
MGSLSLFKSQLEILMLLLSLSK

SEQ ID NO: 70 - protein, 20 aa, Arabidopsis thaliana
MSVYIHVPISLNCFSPKSSC

SEQ ID NO: 71 - protein, 11 aa, Arabidopsis thaliana
MGVPNFRPRNR

SEQ ID NO: 72 - protein, 23 aa, Arabidopsis cebennensis
MRSRVSFFFFKIMLFRLLGYRSM

SEQ ID NO: 73 - protein, 44 aa, Arabidopsis cebennensis
MHTYIHTISNISSIFFCSKRSFSPFTYIRIIVVIDPFRIALTFR

SEQ ID NO: 74 - protein, 22 aa, Arabidopsis halleri
MRSRVSLFLSFSSNFAAYSPRS

SEQ ID NO: 75 - protein, 48 aa, Arabidospis lyrata
MHTYIPSSSFPISNISSVFFCYKRSFSPYTYIRIIVVIDPFRIALTFR

SEQ ID NO: 76 - protein, 50 aa, Arabidopsis thaliana
MNIHTYHHLLFPSLVFHQSSDVPNALSLHIHTYEYIIVVIDPFRITLAFR

SEQ ID NO: 77 - protein, 19 aa, Arabidopsis thaliana
MFQTLYLFIYIHTNILLLS

SEQ ID NO: 78 - protein, 45 aa, Brassica rapa
MFKLYFSAILSTQYMHTYHHRIALIFLSILYPSTNYLMSPILNPT

SEQ ID NO: 79 - protein, 20 aa, Carica papaya
MKIKLGFSLIKIIILLDKNS

SEQ ID NO: 80 - protein, 21 aa, Capsella rubella
MHPHTYIHIPSSSFLISSFCL

SEQ ID NO: 81 - protein, 45 aa, Eucalyptus grandis
MKHIQRWRYGETSGRQGDWKRLEIKVHSNPSLKVKKNTNNFSSSL

SEQ ID NO: 82 - protein, 28 aa, Gossypium raimondii
MIHFNLSQWRAICMANFHLTYSFLFGVL

SEQ ID NO: 83 - protein, 21 aa, Medicago truncatula
MHVYLELFMVIKGLGFLLLVK

SEQ ID NO: 84 - protein, 23 aa, Oryza sativa
MEMIQRPCLILKFFFKLSTLYIP

SEQ ID NO: 85 - protein, 38 aa, Physcomitrella patens
MFHRRRSSVLLPPFGQTQPNPRCLPDLRFPSCFTPCTA

SEQ ID NO: 86 - protein, 42 aa, Thellungiella halophila
MTICKVSKACFYAGKIENSRLIKKIGIPKREGAPFSPIRENQ

SEQ ID NO: 87 - protein, 37 aa, Thellungiella halophila
MEIQIKKKNLYIMNTQKLPNLYIYIYKYVFIKLMVVE

SEQ ID NO: 88 - protein, 43 aa, Arabidopsis thaliana
MVPQINLWSSRVILKIRIDSSTHREEDHCIQNHKHGLSFIFSF

SEQ ID NO: 89 - protein, 16 aa, Arabidopsis thaliana
MSLQFYERVSFKNTVK

SEQ ID NO: 90 - protein, 12 aa, Arabidopsis thaliana
MTEQEEESQMST

SEQ ID NO: 91 - protein, 39 aa, Arabidopsis thaliana
MYLQYIDNVISIYSNNRRVGRMFSRVPLSTSLEIQFFIK

SEQ ID NO: 92 - protein, 12 aa, Arabidopsis thaliana
MSKEIFFSPGFE

SEQ ID NO: 93 - protein, 44 aa, Arabidopsis thaliana
MRTHEQSTAITTLRHCYSSRFMCSQVTPAELFLYRPCFINAVAR

SEQ ID NO: 94 - protein, 5 aa, Arabidopsis thaliana
MKRNM

SEQ ID NO: 95 - protein, 5 aa, Arabidopsis thaliana
MQCEI

SEQ ID NO: 96 - protein, 4 aa, Arabidopsis thaliana
MFCA

SEQ ID NO: 97 - protein, 6 aa, Arabidopsis thaliana
MVMAHH

SEQ ID NO: 98 - protein, 54 aa, Arabidopsis thaliana
MMKPRWNCSLYGITEWTNNQNQKSKRKGRRKTQIWRIGDRLDTVECITLMLSAY

SEQ ID NO: 99 - protein, 10 aa, Arabidopsis thaliana
MLLIIVELVL

SEQ ID NO: 100 - protein, 14 aa, Arabidopsis thaliana
MLCFNFRCVRRFAE

SEQ ID NO: 101 - protein, 36 aa, Arabidopsis thaliana
MYTYQLDNSFSWFLCTRFCLYRYFLFNFRCFRRFSE

SEQ ID NO: 102 - protein, 88 aa, Drosophila melanogaster
MWREVCAQKSQTKRRNFITGNQRRNKTKANRKAETKQQKVYEFFVQARERCKTRKKHEKKTLKKTKKIQNRYRAVSENEWGKGFPSHI

SEQ ID NO: 103 - protein, 36 aa, Drosophila melanogaster
MRTKKSNKKAQFYYGQPTTKQNKSQPKSRNKAAKSL

SEQ ID NO: 104 - protein, 71 aa, Drosophila melanogaster
MEPGFVFVLFPTHLSTQHTQREKSILVMGLNLQSAKQSDKQNSKERKKNTQINSQRIPYRQGGQCSKVLSP

SEQ ID NO: 105 - DNA, 92 bp, Arabidopsis thaliana
atgttctgttcaattcaatgcgtcgccagacatctgttccctttgcatgtaagagagataaagaaagcgacaagagccataaagaaaggtaa

SEQ ID NO: 106 - DNA, 75 bp, Arabidopsis thaliana
atgcgtcgccagacatctgttccctttgcatgtaagagagataaagaaagcgacaagagccataaagaaaggtaa

SEQ ID NO: 107 - DNA, 114 bp, Arabidopsis thaliana
atggttatgttttttctcgatttagacaaaaaccctagatttgatcttctaaagggtctcaaatggaatctcttctcttctcatatctctccctctctccctccctctctttga

SEQ ID NO: 108 - DNA, 36 bp, Arabidopsis thaliana
atgaaggacaactttcctcttctccttcggttataa

SEQ ID NO: 109 - DNA, 15 bp, Arabidopsis thaliana
atgagtgatgactga

SEQ ID NO: 110 - DNA, 51 bp, Arabidopsis thaliana
atgatatatataaataaatatgggtcgatatcggctgtggaggacgactag

SEQ ID NO: 111 - DNA, 15 bp, Arabidopsis thaliana
atgagccaaagataa

SEQ ID NO: 112 - DNA, 51 bp, Arabidopsis lyrata
atgacgtgtcctcttctctctctctctttccttctctctaagtatatttag

SEQ ID NO: 113 - DNA, 51 bp, Arabidopsis thaliana
atgacgtggcctcttctctctctctctttccttctctctaagtatgtttag

SEQ ID NO: 114 - DNA, 53 bp, Capsella rubella
atgacgtgtactctctctgctctatctctctctctaaatatgtttagggttaa

SEQ ID NO: 115 - DNA, 18 bp, Arabidopsis thaliana
atgttttatctttcataa

SEQ ID NO: 116 - DNA, 114 bp, Arabidopsis thaliana
atggttaatactagtagctttttcatttcaagttttatccttccattggttctttctgagtcaaattgtctcctgtttcgaaccatatataagttttcaatggttttgtattaa

SEQ ID NO: 117 - DNA, 75 bp, Arabidopsis thaliana
atgttttgtttgttgattcccatcttctcttttgtcttttcaccaaatcgtcatttaaggcttcaagaacagtaa

SEQ ID NO: 118 - DNA, 18 bp, Arabidopsis thaliana
atgttttcccctcaatga

SEQ ID NO: 119 - DNA, 72 bp, Arabidopsis thaliana
atgaaatacatacacattttgattttatttaaatcaagatcgacgtataagctatccaccaatcatatttaa

SEQ ID NO: 120 - DNA, 33 bp, Arabidopsis thaliana
atgaaaattccattgtttctgccgaagctttga

SEQ ID NO: 121 - DNA, 84 bp, Arabidopsis thaliana
atggtatctggtcaagaagattcctggttaaaactttcatctctctgtttcctttttctttctttgttggattcattaatttga

SEQ ID NO: 122 - DNA, 105 bp, Arabidopsis thaliana
atgtttcttttaatctttttgagattaataatgatttgtgtttgttcatcaaccgattttctcagatctgtcaattatttttgtttatttatttatgatttatga

SEQ ID NO: 123 - DNA, 30 bp, Arabidopsis thaliana
atgtccactactcaagagcataggtcttga

SEQ ID NO: 124 - DNA, 78 bp, Arabidopsis thaliana
atgatactaaagtgctggagttcccggttcctgagagtgagtccatatcaaaatgcgcattcgttatcacttggttga

SEQ ID NO: 125 - DNA, 42 bp, Arabidopsis lyrata
atgcccttagcagttattagacaagggattgtttggccctag

SEQ ID NO: 126 - DNA, 75 bp, Arabidopsis lyrata
atgccatcatggcatgacatggttcttttgccttacgtaaaacacactcacgccaacacacgccacataacataa

SEQ ID NO: 127 - DNA, 27 bp, Arabidopsis lyrata
atgacatggttcttttgccttacgtaa

SEQ ID NO: 128 - DNA, 114 bp, Arabidopsis thaliana
atgccatcatggcatggtatggttcttttgccttacgtaaaacacactcacgccagcacacacacacacacacataacatatacggatgtgcgtgtgagctagtcttccattaa

SEQ ID NO: 129 - DNA, 69 bp, Arabidopsis thaliana
atggcatggtatggttcttttgccttacgtaaaacacactcacgccagcacacacacacacacacataa

SEQ ID NO: 130 - DNA, 27 bp, Arabidopsis thaliana
atggtatggttcttttgccttacgtaa

SEQ ID NO: 131 - DNA, 24 bp, Brassica rapa
atgatgataattttgtggaaataa

SEQ ID NO: 132 - DNA, 75 bp, Brassica rapa
atgctttgggccaagctagtttcttttagcactcttcactcactagtttttcttctcagcccttcttttgcgtga

SEQ ID NO: 133 - DNA, 120 bp, Brassica rapa
atgccatcatggcatggcattgtcattttgcctttcgtaaaacacactcacgccaacatacattattcatattcatgtgtatgtatatgaatgccatcatggcatatgccatcatggcat

SEQ ID NO: 134 - DNA, 105 bp, Carica papaya
atgattgcatgccatccctacttgccttttccccttttcctttctctaacattttactcaatcttcttctccccctcccccccttccccctctctgccattataa

SEQ ID NO: 135 - DNA, 162 bp, Carica papaya
atgccatccctacttgccttttccccttttcctttctctaacattttactcaatcttcttctccccctcccccccttccccctctctgccattataaccataattaaacctctctccctctctctccctctctctctctctctctctgggttctcagtataa

SEQ ID NO: 136 - DNA, 48 bp, Capsella rubella
atggaattaaaaggtttgagaacttggcagttattagacaaggtatag

SEQ ID NO: 137 - DNA, 45 bp, Capsella rubella
atgccatcatggcatggcatggcatgtttctattgccttacgtaa

SEQ ID NO: 138 - DNA, 90 bp, Capsella rubella
atggcatggcatgtttctattgccttacgtaaaacacactcacgccaacacatactcactatacatgtaaataagtatgtgcgcgtgtga

SEQ ID NO: 139 - DNA, 108 bp, Gossypium raimondii
atgatgagatcaagaattttaaagtttcaatatagatttggcatgggtattggcggcagaaagcaattaaaaaaccagttatgtcaaattcaaggtcgtatcagttaa

SEQ ID NO: 140 - DNA, 33 bp, Gossypium raimondii
atgtcaaattcaaggtcgtatcagttaaaatga

SEQ ID NO: 141 - DNA, 54 bp, Gossypium raimondii
atgaatgaagatttagaaatttcaacaaggaagaggaccccacagctttgttaa

SEQ ID NO: 142 - DNA, 39 bp, Medicago truncatula
atgcccaaatttgatatttttttttatatatttgtatag

SEQ ID NO: 143 - DNA, 231 bp, Medicago truncatula
atgtcatatatctctctctctcctaagttgctacctataaatactaagcctttcccttggttggttcaattcaacttctacttctcatcaaacacaaagtgcaataagcttcatttcctgggtgagaagctccttgttggagaagcagggcacgtgcaaatcctctttctgattcattctctcataatgcatatcaatatcttttgcacgtgctccccttctccaactagg

SEQ ID NO: 144 - DNA, 63 bp, Oryza sativa
atgcaaacccactccaacactccacaatccacatactctctctctctctctctctctgagtag

SEQ ID NO: 145 - DNA, 48 bp, Oryza sativa
atgtgtgtgtgtgatatcaatatgcattcgatgttgatgctactgtag

SEQ ID NO: 146 - DNA, 78 bp, Arabidopsis lyrata
atgagaattaagctatttcagttgaggggaatgttgtctggatcgaggatattatacatatatacatgtgtatgttga

SEQ ID NO: 147 - DNA, 57 bp, Arabidopsis thaliana
atgagggttaagctatttcagttgaggggaatgttgtctggatcgaggatattatag

SEQ ID NO: 148 - DNA, 111 bp, Brassica carinata
atgagaatgaagctatttcagttgaggggaatgttgtctggatcgaggatattatatatacacaaatacgtatatatgttaatacaagtgtttgatcatatatgtatatag

SEQ ID NO: 149 - DNA, 84 bp, Brassica juncea
atgagaatgaagctatttcagttgaggggaatgttgtctggatcgaggatattatatatacacaaatatgtatatatatgttaa

SEQ ID NO: 150 - DNA, 111 bp, Brassica napus
atgagaatgaagctatttcagttgaggggaatgttgtctggatcgaggatattatatatacacaaatacgtatatatgataatacaagtgtttgatcatatatgtatatag

SEQ ID NO: 151 - DNA, 111 bp, Brassica oleracea
atgagaatgaagctatttcagttgaggggaatgttgtctggatcgaggatattatatatacacaagtacgtatatatgttaatacaagtgtttgatcatatatgtatatag

SEQ ID NO: 152 - DNA, 84 bp, Brassica rapa; identical to SEQ ID NO: 149

SEQ ID NO: 153 - DNA, 60 bp, Arabidopsis thaliana
atgttggatctctttcgatctaacaatcgaattgaaccttcagatttcagatttgattag

SEQ ID NO: 154 - DNA, 15 bp, Arabidopsis thaliana
atgagagatagataa

SEQ ID NO: 155 - DNA, 33 bp, Arabidopsis thaliana
atgaacagaaaaatctctctttctctttcttga

SEQ ID NO: 156 - DNA, 27 bp, Arabidopsis thaliana
atgatgggttgttttgtgggattttaa

SEQ ID NO: 157 - DNA, 27 bp, Arabidopsis thaliana
atgcaggaggaaacatatgaggggtga

SEQ ID NO: 158 - DNA, 180 bp, Arabidopsis thaliana
atgccacatacaaacttgaaagatctcttcatcttttctccaaatgtttttttttcgtttgctatttatctccacaattcttggaacaaaaactacattcacaaacgagagaattttcacaacacctcttttgctctcattttttttttttcgtccattatgagtattaattatggttag

SEQ ID NO: 159 - DNA, 120 bp, Arabidopsis thaliana
atgtttttttttcgtttgctatttatctccacaattcttggaacaaaaactacattcacaaacgagagaattttcacaacacctcttttgctctcattttttttttttcgtccattatga

SEQ ID NO: 160 - DNA, 21 bp, Arabidopsis thaliana
atgagacataaagagagttaa

SEQ ID NO: 161 - DNA, 105 bp, Arabidopsis thaliana
atgaacctcctcaagaaggaaagacagaggaggagacaaagaagtataggttcacattgcatagccagtttagttttgaaggatggatatatgaaaaaaatatga

SEQ ID NO: 162 - DNA, 30 bp, Arabidopsis thaliana
atggttctctccggtaaattaacattttag

SEQ ID NO: 163 - DNA, 63 bp, Medicago truncatula
atgcttcttcataggctctccaaattttgcaaaattgaaagagacatagtatatatatcttag

SEQ ID NO: 164 - DNA, 18 bp, Medicago truncatula
atgaagattgaagagtaa

SEQ ID NO: 165 - DNA, 105 bp, Zea mays
atgcatctgccttcaactccctctcgccccccaccccaacacacatctctctcttttctagggaaggaaatgacgaaggggacgacgacggcatgcttcggctag

SEQ ID NO: 166 - DNA, 33 bp, Arabidopsis thaliana
atgttgtctctttctcattttcatatctgctaa

SEQ ID NO: 167 - DNA, 72 bp, Medicago truncatula
atgatggtgtttgggaagccgaaaaaagcgatgttggtgaggttcaatccgaagacggatttacatgtatag

SEQ ID NO: 168 - DNA, 33 bp, Medicago truncatula
atggcttcagctgcaaaagtatacatggcgtga

SEQ ID NO: 169 - DNA, 21 bp, Arabidopsis thaliana
atggcttccaagatctggtaa

SEQ ID NO: 170 - DNA, 33 bp, Arabidopsis thaliana
atggttaggttccaactaagtatacgagattaa

SEQ ID NO: 171 - DNA, 39 bp, Arabidopsis thaliana
atgtgtacgtactattatctcataaataaatatttttaa

SEQ ID NO: 172 - DNA, 36 bp, Arabidopsis thaliana
atgtttccagcaaaatggtgccgtcttgagtcttga

SEQ ID NO: 173 - DNA, 69 bp, Arabidopsis thaliana
atgggatctctctctttatttaaaagtcaattagagatcttgatgctacttctgtccctttccaagtga

SEQ ID NO: 174 - DNA, 63 bp, Arabidopsis thaliana
atgagtgtatatattcatgtacctatctctctcaattgcttctcaccaaaatcatcttgctga

SEQ ID NO: 175 - DNA, 36 bp, Arabidopsis thaliana
atgggagttcccaactttagacctcgaaaccgataa

SEQ ID NO: 176 - DNA, 72 bp, Arabidopsis cebennensis
atgagatctagggtttctttctttttcttcaaaatcatgctttttcgcttgctaggttatagatccatgtaa

SEQ ID NO: 177 - DNA, 134 bp, Arabidopsis cebennensis
atgcatacatacatacataccatctctaatatttcatcaatcttcttttgttccaaacgcctttctctccatttacatacatacgaatcattgttgtcatagatccgtttagaattgctttaacttttagatga

SEQ ID NO: 178 - DNA, 69 bp, Arabidopsis halleri
atgagatctagggtttctttgtttctttcgttttcttcaaattttgctgcatattctccaagatcatga

SEQ ID NO: 179 - DNA, 147 bp, Arabidospis lyrata
atgcatacatacataccatcatcatcttttcccatctctaatatttcatcagtcttcttttgttacaaacgctctttctcgccatatacatacataagaatcattgttgtcatagatccgtttagaattgctttaacttttagatga

SEQ ID NO: 180 - DNA, 153 bp, Arabidopsis thaliana
atgaatatacatacataccatcatcttcttttcccatctctagtttttcatcaatcttctgatgttccaaacgctctatctcttcatatacatacatacgaatatattattgttgtcatagatccatttagaatcactttagcttttagatga

SEQ ID NO: 181 - DNA, 60 bp, Arabidopsis thaliana
atgttccaaacgctctatctcttcatatacatacatacgaatatattattgttgtcatag

SEQ ID NO: 182 - DNA, 138 bp, Brassica rapa
atgtttaagctctacttctcagcaattctctccacccaatacatgcatacataccatcatcgtatcgctctaatttttctatcaatcttgtatccttccacaaattatcttatgtctcccattttaaatcctacatag

SEQ ID NO: 183 - DNA, 63 bp, Carica papaya
atgaagattaaattaggttttagtcttattaagattattatattactagacaaaaacagttaa

SEQ ID NO: 184 - DNA, 66 bp, Capsella rubella
atgcatccacatacatacatacatataccatcatcttcttttctcatctctagtttttgtttataa

SEQ ID NO: 185 - DNA, 138 bp, Eucalyptus grandis
atgaagcatattcaaaggtggagatatggggagacttccggaaggcaaggggattggaaaaggctcgagatcaaagtgcatagcaacccttcgctaaaggtgaaaaagaatacgaataacttcagtagctcactttaa

SEQ ID NO: 186 - DNA, 87 bp, Gossypium raimondii
atgatccatttcaacctgtcacagtggagagcaatttgtatggctaatttccatctcacctattcttttctgtttggggttctctag

SEQ ID NO: 187 - DNA, 66 bp, Medicago truncatula
atgcatgtatatcttgaattgtttatggtaataaaggggttaggatttctccttttggtgaagtga

SEQ ID NO: 188 - DNA, 72 bp, Oryza sativa
atggaaatgatacaaaggccgtgtttaattttaaaattttttttcaaactttcaacactttacatcccataa

SEQ ID NO: 189 - DNA, 117 bp, Physcomitrella patens
atgttccaccgtcggagatcctcggtgctgctacccccgttcggccaaacccaacccaaccctaggtgtctgccggacctccgcttcccctcctgcttcaccccctgcaccgcttaa

SEQ ID NO: 190 - DNA, 129 bp, Thellungiella halophila
atgacgatatgtaaagtaagcaaggcatgtttttatgcagggaagattgaaaattcaagattaatcaagaaaattggaataccaaaaagagagggagctcccttcagtccaatcagagagaatcaatga

SEQ ID NO: 191 - DNA, 114 bp, Thellungiella halophila
atggagattcaaattaaaaagaaaaacttatatataatgaatacacaaaagctacctaatctgtatatatatatatataaatatgtcttcattaaattaatggtcgtggaatag

SEQ ID NO: 192 - DNA, 132 bp, Arabidopsis thaliana
atggtacctcaaattaatctatggtcatctagggttatcttgaagattagaattgattctagcacgcacagagaggaagatcattgcatccagaatcacaaacatggcctatcttttatcttttctttttga

SEQ ID NO: 193 - DNA, 51 bp, Arabidopsis thaliana
atgtctctccaattttatgagagggtttccttcaagaacacagtaaaatag

SEQ ID NO: 194 - DNA, 39 bp, Arabidopsis thaliana
atgacagagcaagaagaagaaagtcaaatgtccacatga

SEQ ID NO: 195 - DNA, 120 bp, Arabidopsis thaliana
atgtatctacaatatattgataatgtaatatctatatattcaaacaatcgtcgtgttggtcggatgttttctagagttcctctgagcacttcattggagatacaattttttataaaatag

SEQ ID NO: 196 - DNA, 39 bp, Arabidopsis thaliana
atgagcaaggagatatttttttcccctgggtttgaatga

SEQ ID NO: 197 - DNA, 133 bp, Arabidopsis thaliana
atgagaacacacgagcaatcaacggctataacgacgctacgtcattgttacagctctcgtttcatgtgttctcaggtcacccctgctgagctctttctctaccgtccatgttttatcaacgccgtggcccgtg

SEQ ID NO: 198 - DNA, 18 bp, Arabidopsis thaliana
atgaagagaaacatgtaa

SEQ ID NO: 199 - DNA, 18 bp, Arabidopsis thaliana
atgcaatgtgaaatatga

SEQ ID NO: 200 - DNA, 15 bp, Arabidopsis thaliana
atgttttgtgcttga

SEQ ID NO: 201 - DNA, 21 bp, Arabidopsis thaliana
atggtcatggctcatcattag

SEQ ID NO: 202 - DNA, 165 bp, Arabidopsis thaliana
atgatgaaacctcgatggaactgctctctttatggaatcacggaatggacaaataatcaaaatcagaaatcgaagcgaaaagggaggagaaaaacgcagatttggaggattggggacagattagatactgttgaatgcatcactctaatgctatcagcctattaa

SEQ ID NO: 203 - DNA, 33 bp, Arabidopsis thaliana
atgctgcttatcatcgtggagttggttctgtaa

SEQ ID NO: 204 - DNA, 45 bp, Arabidopsis thaliana
atgctttgtttcaatttcaggtgcgttagaaggtttgcagagtag

SEQ ID NO: 205 - DNA, 108 bp, Arabidopsis thaliana
atgtacacctaccagcttgataactctttttcgtggtttctgtgtactcgtttctgtttgtacagatacttcttgttcaatttcagatgctttagaaggttttcggag

SEQ ID NO: 206 - DNA, 267 bp, Drosophila melanogaster
atgtggcgcgaagtatgcgcacaaaaaagtcaaacaaaaaggcgcaattttattacgggcaaccaacgacgaaacaaaacaaaagccaaccgaaaagcagaaacaaagcagcaaaaagtttatgaattttttgtgcaggcgcgtgaaagatgcaaaacgagaaaaaaacatgaaaaaaaaacattaaaaaaaacaaaaaaaatccaaaacagataccgagctgtatccgaaaacgagtggggaaaggggtttcccagtcacatataa

SEQ ID NO: 207 - DNA, 111 bp, Drosophila melanogaster
atgcgcacaaaaaagtcaaacaaaaaggcgcaattttattacgggcaaccaacgacgaaacaaaacaaaagccaaccgaaaagcagaaacaaagcagcaaaaagtttatga

SEQ ID NO: 208 - DNA, 216 bp, Drosophila melanogaster
atggagcctggctttgtttttgttttatttccaacccacttgagcacacagcacacacagagagaaaaatcaatactcgttatgggattaaatttacaaagcgcaaagcaaagcgacaaacaaaattcaaaagaaagaaaaaaaaacactcaaataaactcacaaagaattccttatcgccaagggggccaatgttctaaggttctttcgccttga

SEQ ID NO: 209 - DNA, 614 bp, Arabidopsis thaliana
attcattgttcactctcaaatctcaagttcattgccatttttaggtctctctataaattcaaatgttctgttcaattcaatgcgtcgccagacatctgttccctttgcatgtaagagagataaagaaagcgacaagagccataaagaaaggtaagactctttgaaatagagagagataaggttttctcttatcttcttctcatcagatctttgtttctttaccctctttctttcttttttttgctttttatggttatgttttttctcgatttagacaaaaaccctagatttgatcttctaaagggtctcaaatggaatctcttctcttctcatatctctccctctctccctccctctctttgattctttgtcttctccagttaaaactcagatctaacacaaagcttaaaagattctcatcgtttcttgttttctttgtttcatcttgtagatctctgaagttggactaattgtgaatgaaagagttgggacaagagaaacgcaaagaaactgacagaagagagtgagcacacaaaggcaatttgcatatcattgcacttgcttctcttgcgtgctcactgctctttctgtcagattccggtgctgatctcttt

SEQ ID NO: 210 - DNA, 422 bp, Arabidopsis thaliana
ctctgcctttagttctttcttttttggtaatatatttatttttcgttacgatttggtcaaaaccctagatttgttttccaaaagcatatctgaaaatgaaggacaactttcctcttctccttcggttataaatattctctccggttttgcttgtttaacctaaaagcctcagatctaactccaacaccttcaaagtctgcctcctttccaatcttctttcttctgttcgatctctaatctcagaatttgtgtcggtaaggtaaaggtgataatgagtgatgactgatgagggagttttgggacaaattttaagagaaacgcatagaaactgacagaagagagtgagcacacaaaggcactttgcatgttcgatgcatttgcttctcttgcgtgctcactgctctatctgtcagattccggct

SEQ ID NO: 211 - DNA, 268 bp, Arabidopsis thaliana
tcccacatccaaagatagaaagatgtaaggtctagagtcttgttcttaatcccctaacagaacaatgatatatataaataaatatgggtcgatatcggctgtggaggacgactagctacggtttcgagcctggtcacatgcgtagagtgtgaaaggtaattaggaggtgacagaagagagtgagcacacatggtggtttcttgcatgcttttttgattagggtttcatgcttgaagctatgtgtgcttactctctctctgtcacccct

SEQ ID NO: 212 - DNA, 328 bp, Arabidopsis thaliana
tcccacagccaatgagccaaagataaagaaacacctatcctataataatttagagcaatatacctccataatggaacatctatatatataaaggtatccgtatatctctatatattatattcattgagtttaaagtggctagggtttatagatgtatgtgatattaagagatatgaaacatatttgtcgacggtttgagtggtgaggaattgatggtgacagaagagagtgagcacacatggtggctttcttgcatatttgaaggttccatgcttgaagctatgtgtgctcactctctatccgtcacccccttctctccctctccctc

SEQ ID NO: 213 - DNA, 592 bp, Arabidopsis lyrata
aaaaaatgacgtgtcctcttctctctctctctttccttctctctaagtatatttagggttaattattagggttctttatctctttcttcagtctttgaagtttcttcaatagctttaattgaagtgatttacctctctgggtgtttttagtatatatatcatgtacatgatcgaatttctttctatccaagttctcatcaaaccttctcatgttttgaagagttaaaggctttatagtttgcttaggtcagatccataacatactgtatttgacaagtttctttgtctcacgatagatcttggtctgaccaaaatgattttctcgagaaaaaaaaagatggaagtagagctccttgaagttcaaacgagagttgagcagggtaaagaaaagctgctaagctatggatcccataagccctaatccttataaagaaaaaaaaggatttggttatatggcttgcatatctcaggagctttaacttgccctttaatggcttttactcttctttggattgaagggagctctacatcttctttcaccttctctatttttctttctttattttctcctctacagtaatttatttggatt

SEQ ID NO: 214 - DNA, 599 bp, Arabidopsis thaliana
ttccaaaacatgacgtggcctcttctctctctctctttccttctctctaagtatgtttagggttaataattagggttcctcctctcttttgttctgtctttatatctccttcatagctctaatgtaagagatttacctcttttggtgtttttgttaatccacgttctcatcaaaactttctcattgttttatgaagagttaaaggtctttacagtttgcttatgtcagatccataatatatttgacaagatactttgtttttcgatagatcttgatctgacgatggaagtagagctccttaaagttcaaacatgagttgagcagggtaaagaaaagctgctaagctatggatcccataagccctaatccttgtaaagtaaaaaaggatttggttatatggattgcatatctcaggagctttaacttgccctttaatggcttttactcttctttggattgaagggagctctacatcttctttcaccttctctattttttatttttctttatttctactcaacaattatttattcggattcatctttaattttccgttataatttctttttggtaaggattattcgctataatttgagaat

SEQ ID NO: 215 - DNA, 623 bp, Capsella rubella
ttccaacgaatgacgtgtactctctctgctctatctctctctctaaatatgtttagggttaattagggttcttcatctgtctctctctctctctctcttcagagtctttatagcttcttccaagatttttaattgaaagtaatttacctcttttggagttctgtacatatagaatatcaggagtcgtgtttcttttttatcaaggttctcatctaacctttatagtattttcattagttgataaaggtcttcatagtttgcttagatcagatcttgtcttcgtcttttcgatagatcttgttctgtccaatatacagtgattttatttcgagagcaaaaaagatgagaggtagagctccttgaagttcaaacgagagtttagcagggtagagaaaagctgctaagctatggatcccataagccctaatccttgttaatgataaaggatttggttatatggcttgcatatctcaggagctttaacttgccctttaattgcttttactcttctttggattgaagggagctctacatcttctttgacttctctctctattaagtctttctttattttcttctctacaatagttgttttggatcggaagatctttaagtttccctta

SEQ ID NO: 216 - DNA, 612 bp, Arabidopsis thaliana
tttcacttttgttctcctcctccctttttttcttttcaggattcttcttttctatgttttatctttcataatagatctgataattttgatttttcactatatatattatggttaatactagtagctttttcatttcaagttttatccttccattggttctttctgagtcaaattgtctcctgtttcgaaccatatataagttttcaatggttttgtattaactcaagtattcaacattatgtctctctttttcttgcttggatctctaatgctgttcatattttaaagcataggtttaggttagatgcatgtaactgccaattaaaagaaggtcaagagttttttgattgtatgaatatatgagttagtcaaagcagatccacacgattatatagaaaaacaaaggaagaagaagaggaagagctccttgaagttcaatggagggtttagcagggtgaagtaaagctgctaagctatggatcccataagccttatcaaattcaatataattgatgataaggttttttttatggatgccatatctcaggagctttcacttacccctttaatggcttcactcttctttggattgaagggagctcttcatctctc

SEQ ID NO: 217 - DNA, 515 bp, Arabidopsis thaliana
catcccacccttaattgttttatataaaccatttctcctcctctctccatcaccttcaatctctctcgatctctctctggatccccaatctcacctccatgttttgtttgttgattcccatcttctcttttgtcttttcaccaaatcgtcatttaaggcttcaagaacagtaaccccaattcctccacaagagggagagaaaacaaaagatcttccaattccattctcgtacatgcaaatcacaatccatgccatagattgtttctattcctccttatttattgcttgtatctgttcatgcatggaccaggtggagagagcattacttaaaaatagaattagctatctgttttaggcgaattagtttccttacataaccatgtatatgtcatgacgcatatacatatgtagatgtatatgtattatatatgtatgcctggctccctgtatgccatatgctgagcccatcgagtatcgatgacctccgtggatggcgtatgaggagccatgcatat

SEQ ID NO: 218 - DNA, 276 bp, Arabidopsis thaliana
actcataactctccccaaattcttgaccaaaaatatccgccactttctctctggttcatgttttcccctcaatgaaatacatacacattttgattttatttaaatcaagatcgacgtataagctatccaccaatcatatttaagggttcccgtatacatatatactatatatatatatggaataatagtcgtgcctggctccctgtatgccacaagaaaacatcgatttagtttcaaaatcgatcactagtggcgtacagagtagtcaagcatgac

SEQ ID NO: 219 - DNA, 243 bp, Arabidopsis thaliana
ctctaactcatccttctcttctatgaaaattccattgtttctgccgaagctttgatcagtacttctcttttgcttgatctcggtttttgaccagtttattgcgtcgatcaatgcattgaaagtgactacatcggggttccgattttttttgttcttcatatgatgaagcggaaacagtaatcaaccctggtttagtcactttcactgcattaatcaatgcatttgtaaaaagagggaaaagca

SEQ ID NO: 220 - DNA, 537 bp, Arabidopsis thaliana
ctagaagaaaaaaccagatctataaagtttgttattaaaagatagagagagaggagggatgtagtaggccaataggcaaatcagagaatcacaaatggtatctggtcaagaagattcctggttaaaactttcatctctctgtttcctttttctttctttgttggattcattaatttgacatatctctatcatcacactgattctctttctcccagtttgtctgcagatgcatgtgtgtaatctagggtatatgtttttgtccatttggtttcataaggcaataaagatccagctatttactacttgtggtatagattttgactgttgaattttcagatctgatgtgtttcgtttgatccgattcggaaaatttatgtttcgttgacattttggagtttagttggaagaagagtgagagtcgctggaggcagcggttcatcgatctcttcctgtgaacacattaaaaatgtaaaagcatgaatagatcgataaacctctgcatccagcgtttgcctcttgtatctttcttattgactt

SEQ ID NO: 221 - DNA, 261 bp, Arabidopsis thaliana
ctgcatctatccacctctctctgtaaatttatctaaatgtttcttttaatctttttgagattaataatgatttgtgtttgttcatcaaccgattttctcagatctgtcaattatttttgtttatttatttatgatttatgaatgaggaaagagtgaagtcgctggaggcagcggttcatcgatcaattcctgtgaatatttatttttgtttacaaaagcaagaatcgatcgataaacctctgcatccagcgctgcttgctc

SEQ ID NO: 222 - DNA, 481 bp, Arabidopsis thaliana
tatcacagttctcatcaaatatttgaaagtatcaaacaaaaaaaggagagtgagaaaaataaagagagagatagagagagatcatgtccactactcaagagcataggtcttgattggtggaagacaagtaccttagataaaccgaccaaaacccggtggataaaatcgagttccaacctcttcaacgacaacgatttcaacactctcttccaggaacaacttcctccaggcagatgatactaaagtgctggagttcccggttcctgagagtgagtccatatcaaaatgcgcattcgttatcacttggttgaacccatttggggatttaaatttggaggtgaaatggaacgcgtaattgatgactcctacgtggaacctcttcttaggaagagcacggtcgaagaagtaactgcgcagtgcttaaatcgtagatgctaaagtcgttgaagaggacttggaacttcgatattatcccccgtgt

SEQ ID NO: 223 - DNA, 471 bp, Arabidopsis lyrata
agtagggttggaaaatttttttacatttttactctaaaatagaatagagttggagatgcccttagcagttattagacaagggattgtttggccctagcgatcctctcttcactctctcacttttgtagttcaacccttcttttgcgtgagatgccatcatggcatgacatggttcttttgccttacgtaaaacacactcacgccaacacacgccacataacataaataaattatatatacatatacgtatgtgcgtgtgagtcttccattaatgcaatctttgggcctatatatatatacaaaccttccataaccaaagttatcatactacaaaagctctctcgtacttggaaatgcgggtgagaatctccatgttggagaagcagggcacgtgcaaaccaacaaacacgaaatccgtctcatgtgttttgcacgtactccccttctccaacatgagctcctgacccattg

SEQ ID NO: 224 - DNA, 466 bp, Arabidopsis thaliana
agacaagcccccacactaaaaaaacagtaatatggaataaaaaaaagctttcaaaacttagcagttattagacaaggtattgtttggccctagctagcgatcgtttagctctcttcactctctcacttttttagttcaacccttcttttgcgtgagatgccatcatggcatggtatggttcttttgccttacgtaaaacacactcacgccagcacacacacacacacacataacatatacggatgtgcgtgtgagctagtcttccattaatgcaatctttgggcctatatatacaaacctttccataaccaaagttctcatactacaaacgcccctcatgtgcttggaaatgcgggtgagaatctccatgttggagaagcagggcacgtgcaaaccaacaaacacgaaatccgtctcatttgcttatttgcacgtacttaacttctccaacatgagctcttcaccc

SEQ ID NO: 225 - DNA, 450 bp, Brassica rapa
agacaaccccacgttttaaaataagaaatgatgataattttgtggaaataaaagctagtatacttttgcaataattagacaaggtattgatgctttgggccaagctagtttcttttagcactcttcactcactagtttttcttctcagcccttcttttgcgtgaaatgccatcatggcatggcattgtcattttgcctttcgtaaaacacactcacgccaacatacattattcatattcatgtgtatgtatatgaatgttccattaatgcaatctttggggcctatatatacgaagcttacatcaccaaagctctcatattacaaaagctcacatatatacttggaaatgtaggtgagaacctccatgttggagaagcagggcacgtgcaaaccaaaaaacatgaaatctgtttcatatgctttgcacgtgctcccctcctccaacatga

SEQ ID NO: 226 - DNA, 513 bp, Carica papaya
agacaacactcctctttgttcccttcctcacgtatccacttttgaaatttgtaatttgtgtgcaccaccatgattgcatgccatccctacttgccttttccccttttcctttctctaacattttactcaatcttcttctccccctcccccccttccccctctctgccattataaccataattaaacctctctccctctctctccctctctctctctctctctctgggttctcagtataaatgcagctctgcttatacttccacacctatatatatatacctgacccttcttcacctccttcatccacctcctccttcttccccaaaactttcttaactgttctctgcatacatatatatccacatacatatatatatatatagagagagagtgagacagagaggttaccgaggcaattgggtgagtagctccctgttggagaagcagggcacgtgcaaattctccatggctttcccctctttgcacgtgctccccttctccaacatgggttcc

SEQ ID NO: 227 - DNA, 464 bp, Capsella rubella
cggccacccccacatttaacaagaaaaaaactgatggaattaaaaggtttgagaacttggcagttattagacaaggtatagtttggccctagcttcttttaatttagctctctccactctcacacttttcaactttcacccttctcttgcgtgagtcgcgagatgccatcatggcatggcatggcatgtttctattgccttacgtaaaacacactcacgccaacacatactcactatacatgtaaataagtatgtgcgcgtgtgagtcttccatccatcaatgcaatctttggggctatatatatacaaaccttttccataaccaaagctctcatataaactacaaaaggctcacttgggaaatgcgggtgagaatctccacgttggagaagcagggcacgtgcaaaccaacaaacacgaaaccctcctcatgtgctttgcacgtactccccttctccaacatg

SEQ ID NO: 228 - DNA, 571 bp, Gossypium raimondii
gaaaacccaagttcaggctaacaagttatctgatgatgagatcaagaattttaaagtttcaatatagatttggcatgggtattggcggcagaaagcaattaaaaaaccagttatgtcaaattcaaggtcgtatcagttaaaatgaatgaagatttagaaatttcaacaaggaagaggaccccacagctttgttaaattaagtgtgtggtttttataattatcatctcgaaagtttcataatatcaattagattaaaacatctctgaatttcataattacaaaccagatagatagatacatgaaaacttagaccccagagatctgtctttaaagaatgcccacttctagactcaatctctattactctctttttttctctctctctctcttcggaaaaacttgtatataaataaatgacactttctttgctttctgcactcaactcatgaacttgaaaagctttacttggatgggttggttgggggtgagtatctcttgttggagaagcagggcacgtgcaagttcctatgtttaagtgaactttgcacgtgctccccttctccaccgtgag

SEQ ID NO: 229 - DNA, 592 bp, Medicago truncatula
gaagagaaaaaacctagtgtaaaatttgatatactctttatgtatagtacgaatgtttttttaaaaattatgtaaaaaatgataaaataataactaactaaattaacagtaaaattagaaaagtaaaatactatgcccaaatttgatatttttttttatatatttgtatagattattattatttgatatgtaaagtccaattaaaaatttgttttaactaagatttgaactaggttttcttaaaagactcatcttttacttcaaatttatttatcatttgaattcaatcactttctaatattattattattatttccaccatactcattgcttctgccacgttactttagttagatctcttatgtcatatatctctctctctcctaagttgctacctataaatactaagcctttcccttggttggttcaattcaacttctacttctcatcaaacacaaagtgcaataagcttcatttcctgggtgagaagctccttgttggagaagcagggcacgtgcaaatcctctttctgattcattctctcataatgcatatcaatatcttttgcacgtgctccccttctccaactagg

SEQ ID NO: 230 - DNA, 520 bp, Oryza sativa
atgcaaacccactccaacactccacaatccacatactctctctctctctctctctctgagtaggagtacatgtgtgtgtgtgatatcaatatgcattcgatgttgatgctactgtagccatcttgtggctatataaacccagcaggcagcagcacagcttagctagagagccatattgcatgcacactcgctaatctcttttctctactctacttgcattacaccacctctgcattgcacttcagttcattcattccactgatgcatggatcgatgttgctaccttcttctcttctcctcatgcatccatgcatcgatctcacctagcttcttcctcatcctctctcgatcgattacaagagaaaagtgtttgctgttcttgctatcgatctacaggtgagtaggttcttgttggagaagcagggtacgtgcaaaatgcacaccggttggtcgagctaattaacaagctctgacgaccatggtgatcgaatgcacgtgctccccttctccaccatggcct

SEQ ID NO: 231 - DNA, 501 bp, Arabidopsis lyrata
ctagggtttaggaatgacgacttgtttctgttgtgtcttattaaaagcccatcttcgtctccgccactcatcattccctcatcataacaccatcatcaccattcaccaacctctctctctttctctctctcctctcgatctacaacaaaatgtgaatctgctaagatcgattatcatgagaattaagctatttcagttgaggggaatgttgtctggatcgaggatattatacatatatacatgtgtatgttgatacatgtgatcatagagagtatcctcggaccaggcttcatcccccccaacatgttattgcctctgatcaccatatatatgtcgttacatttcatggttaattacttgcacaaatcacaaaagcttggtttgtaactttctatgaccttttttaatgactttgaatctttcatgcatgacttcttaagagtagatttacacatttgcggatccgtttatgctttttgcttttgtttcgtttatatatat

SEQ ID NO: 232 - DNA, 484 bp, Arabidopsis thaliana
ctagggtttaggaatgacgacctgtttctgttgtgtcttattaaaagcccatcttcgtctccgccactcatcattccctcatcataacaccatcatcaccattcaccaacctctctctctctctcctctatcactctctacaacaaaaatttgtgaatctgctaagatcgattatcatgagggttaagctatttcagttgaggggaatgttgtctggatcgaggatattatagatatatacatgtgtatgttaatgattcaagtgatcatagagagtatcctcggaccaggcttcatcccccccaacatgttattgcctctgatcaccatttattgttacatttttttttgttaattacttgcgcaaattacaaaagcttggtttttgtgatgactttgaatctttcttgcatggcttcttaagagtagatttacggatccgtctatgctttttgctttttgtttcgtttatttgtatttaaac

SEQ ID NO: 233 - DNA, 552 bp, Brassica carinata
gagatcaatgaaattatcctgccaaataaaacgtgtgacgtttattcaaaaatatatgcattagatgctttgatattaaaatatttccttttaaaagctagctagggtttaggaatgacgagttgtgtcttattaaaagcccttcttctcctccgccactcatcattccctcatcataacaccatcatcaccattcacccacctctcctctttctctctctctctctctctctctctctctagaacaacaagtgagaatctgctaaaatattgtgactattatcatgagaatgaagctatttcagttgaggggaatgttgtctggatcgaggatattatatatacacaaatacgtatatatgttaatacaagtgtttgatcatatatgtatatagattattctcggaccaggcttcatcccccctaacatgttattgcctctgatcaccagattctatcaactcttcgcttattattttgtcacaaacaagtaataagctcataattttctttgagtctttcagcatcgtttcattatgtttttcgaatccg

SEQ ID NO: 234 - DNA, 566 bp, Brassica juncea
gagatcaatgaaattatcctgccaaataaaacgtgtgacgtttattcaaaaatatatgcattaaatgctttgatattaaaatatttccttttaaaagctagctagggtttaggaatgacgagttgtgtcttattaaaagcccttcttctcctccgccactcatcattccctcatcataacaccatcatcaccattcatccacctcttctctcctctctctctctctctctctctctctctctctctctctctctagaacaacaagtgagaatctgctaaaatattgtgattattatcatgagaatgaagctatttcagttgaggggaatgttgtctggatcgaggatattatatatacacaaatatgtatatatatgttaatatcagtgtttgatcatatatatgtatatagattattctcggaccaggcttcatcccccctaacatgttattgcctctgatcaccagattctatcaactcttagcttattatttgtcacaaacaagtaataagctcaataatgtctttgagtctttcagcatcgtttcatatgttttcgaatccg

SEQ ID NO: 235 - DNA, 549 bp, Brassica napus
gatatcaatgaaattatcctgccaaataaaacgtgtgacgtttattcaaaaatatatgctttaaatgctttcatattaaaatatttccttttaaaagctagctagggtttaggaatgacgagttgtgtcttattaaaagcccttcttctcctccgccactcatcattccctcatcataacaccatcatcaccattcacccacctctcctctttctctctctctctctctctctctctctctagaacaacaagtgagaatctgctaaaatattgtgactattatcatgagaatgaagctatttcagttgaggggaatgttgtctggatcgaggatattatatatacacaaatacgtatatatgataatacaagtgtttgatcatatatgtatatagattattctcggaccaggcttcatcccccctaacatgttattgcctctgatcaccagattctatcaactcttcgcttattatttgtcacaaacaagtaataagctcaataatgtctttgagtctttcagcatcgtttcatatgttttcgaatccg

SEQ ID NO: 236 - DNA, 543 bp, Brassica oleracea
gggatcaatgaaaattatcctgccaaataaaaacgtgtgacgtttatccaaaaatatatgcattaaatgctgtgatatgaagtatttcctttaaaagctagctagggtttaggaattacgagttgtgttttattaaaagcccttcttctcctccgccactcatcattccctcatcataacaccatcatcaccattcacccacctctcctctttctctctctctctctctctctctagaacaacaagtgagaatctgctaaaatattgtgactattatcatgagaatgaagctatttcagttgaggggaatgttgtctggatcgaggatattatatatacacaagtacgtatatatgttaatacaagtgtttgatcatatatgtatatagattattctcggaccaggcttcatcccccctaacatgttattgcctctgatcaccagattctatcaactcttcgcttattatttgtcacaaacaagtagtaagctcaataatgtctttgagcctttcagcatcgtttcatatgttttcgaatccg

SEQ ID NO: 237 - DNA, 566 bp, Brassica rapa; identical to SEQ ID NO: 234

SEQ ID NO: 238 - DNA, 414 bp, Arabidopsis thaliana
catcatcaccactcacttatcttcttctccatctctctctctgcttctcccttaatcttagccgggtctcgtgggggacgaacatagaaagagagagatataaagatatatattcagaaaccctagattctataatttcgactgaaaagaaaaaggggctttctcttttgaggggactgttgtctggctcgaggactctggctcgctctattcatgttggatctctttcgatctaacaatcgaattgaaccttcagatttcagatttgattagggttttagcgtcttcggaccaggcttcattccccccaattgttgctccctgtttactccatatttcttccttcttttcaaattagggtttcagatccagtgaatgaacccttgttaaaggtttgatctcttaccttacttt

SEQ ID NO: 239 - DNA, 328 bp, Arabidopsis thaliana
tctcatcattctcttcatcatcaccacattcatctctctctctctctctctctctctctctttctcttccttgatcttagccggatctgttgggggacgaacacatgagagatagataaaatataagaaatttctcgaaaaaacctaatagaaaaaggtctgtttcttaaagaagaagaagaagaggatttaaagagggatttttcttttgaggggactgttgtctggctcgaggactcttattctaatacaatctcatttgaatacattcagatctgatgattgattagggttttagtgtcgtcggaccaggcttcattccccccaa

SEQ ID NO: 240 - DNA, 192 bp, Arabidopsis thaliana
tgatgaacagaaaaatctctctttctctttcttgatctgctacggtgaagtctatggtgcaccggcatctgatgaagctgccagcatgatctaattagctttctttatcctttgttgtgtttcatgacgatggttaagagatcagtctcgattagatcatgttcgcagtttcacccgttgactgtcgcaccc

SEQ ID NO: 241 - DNA, 846 bp, Arabidopsis thaliana
aaccacaaagtaccgctgctattttctttttacgtctttgtatttgcatcgtctaagagaatgatgggttgttttgtgggattttaatgcaggaggaaacatatgaggggtgattaaggcaaaaaccttaagatgtggtcatttagatacatggagtcaaactaagaatggaccttggcgaaagcttcttcacggtcaagatttaaaatcaggtacgacactgtgtacgtgagagagagagagagagagagaaagagattatagaaagaaagagatgtatcacaataaaggagtatatttagggtcacaggtggtggagatataggtatgcagggccaaggctctaatctcttcatagccctattgattttgtccctctctctctctctttcttcctctcttagctgtatgcattatgatgcgtcttttaattcactgtttcaggcttctttaattcgtggtgtctctctcctttttacccaaccatctcttaaaatttttaacatctgttcctcaaatcctctctcatctctttctataagtatctatagcgcctcttaaaccacaaagcatcacctctgtcttctctcatctcctttctgtattctctttcattgccttcacgtctgttgcaatttctccacttcttgagcttccgttttttacaattattgatccgtcaaatatgtgagatttgcacaacttgttgctcaggtattttgaagacaagtccacaagggaacaagtgaagctgccagcatgatctatctttggttaagagatgaatgtggaaacatattgcttaaacccaagctaggtcatgctctgacagcctcactccttcct

SEQ ID NO: 242 - DNA, 571 bp, Arabidopsis thaliana
gagcaagacaatgccacatacaaacttgaaagatctcttcatcttttctccaaatgtttttttttcgtttgctatttatctccacaattcttggaacaaaaactacattcacaaacgagagaattttcacaacacctcttttgctctcattttttttttttcgtccattatgagtattaattatggttagggaatcttacagaatgaaaatgaaggtgtgaatggattgtctcatctaaagccttgaatgtgggaaaaaggccattgttgttcagccaaggatgacttgccggtagcttgtattatgattactctatattcgatttatattatggagatgatggtttatatatatttacttatctacatagttttagttgattttttttcgtacgtaatataatacgaaaaagtatttacttatttatatatgtgtgttggggcaagaagtgtaaccaagctagcccggcaagtcatctatggctatgcaactgtctcttcctctcattctaggcttacgatgacacgtaaaaaatcccaaatatcactaatatgatatgaatatggatga

SEQ ID NO: 243 - DNA, 241 bp, Arabidopsis thaliana
aggcatgagacataaagagagttaaatataatgaagaagagaggtctaatatggcgaaaagagtcatgtttaatagccaaggatgacttgcctgatctttttcacctccatgattcaattttaagttcgtggattttggattattatgcgtttaaaaggtataataatttgagatcatgttgaatcttgcgggttaggtttcaggcagtctctttggctatcttgacatgctttcttcatc

SEQ ID NO: 244 - DNA, 689 bp, Arabidopsis thaliana
gaattttgatttatgaacctcctcaagaaggaaagacagaggaggagacaaagaagtataggttcacattgcatagccagtttagttttgaaggatggatatatgaaaaaaatatgaagagagagaagagagaagaagaggaggattaaagagggtgaggccagcttttgtgctttggtagtagatgaggtttaaatgctccataccttccatttccttctctcttaccctaatttaattcttcctctcctttataactccccacagacattctcacttctcctcctcacacttcacatcaacacttctttcttgttttttcattttacaatgtttcctttgatatccgcactttaagcatgagagagtccctttgatattggcctggttcactcagatcttacctgaccacacacgtagatatacattattctctctagattatctgattgagccgcgccaatatctcagtactctctcgtctctattttggactttgtggtcttgtagatcgatttgtatgtgtgtgttgaaatggagacaagtacttgtaacttctttgttgttatattgtttacctataggctgatgtcataaactcttttgatcttgtttctaacttccagattcttgaaaaatcaagtcgtgtgtgtgtctccatggaagccttttccatttcttcctttcca

SEQ ID NO: 245 - DNA, 452 bp, Arabidopsis thaliana
actcataaactttgctactggccgcatttctattttctccttcgattcttctaattcgtactttggtttctgacgtccctaaaatttttagacagtaagagtttctccaggatccgatggttctctccggtaaattaacattttagtgtcaatagtcatttatacatatttttatttcactttttgttttgtttattggttttctggagctaagtggagattatagtcgaacaagagtggttttatgcaaggtaacgcgagatattagtgcggttcaatcaaatagtcgtcctcttaactcatggagaacggtgttgttcgattgagccgtgccaatatcacgcggtaaaccaaaaatggcaaagatagttattataaccttaaaggtatgtatcattatcgttttattgtttcaattttgattaatggctttgatatttcatttttttttt

SEQ ID NO: 246 - DNA, 767 bp, Medicago truncatula
attggtcaaacatacatacagtagcactagctggtttcattattccactatgcttcttcataggctctccaaattttgcaaaattgaaagagacatagtatatatatcttagcaaggagaaattcaggatattgaggatgaagattgaagagtaatcagtgatgaagaaagcaagcaaggtattggcgcgcctcaatttgaatacatggctataaaaatgcatcatatcagccatgtagtttgattgagccgcgtcaatatcttgtttccatctccaaatttaccaatctcatcaaatcaaattaacaccacaatcaaggctttcatttaatgcagtcaaaataggttgaccttatcatcgaagaaattgttttctcattcctatcgaagttggacttgccgaaaatgctcgaaagcatgtgttttagttcgacaggcgaaaaagttaccgaaggacaatttggttgtggttcggataagatcaagcaacggatattttcaagacacgttcgaaattcaaatcaaatggataagtatcgttagtttactgcagttatagttttaaattcaaatctaggcagttgtttctatttgtataaatagtagtttttccctagggaaaaggggtcgcaattcaatcatacaaaaaacttacaatcaaattatccgcatggaagagagaaacgagtcacaagttgcaatgtatgaacatgtgtaccaatttacattcaatcagtacaatttaagttcatttccataaaaaaaaa

SEQ ID NO: 247 - DNA, 854 bp, Zea mays
accagggttaggtatccatccacacagcaatgcatctgccttcaactccctctcgccccccaccccaacacacatctctctcttttctagggaaggaaatgacgaaggggacgacgacggcatgcttcggctagctcgttggtgctaggacaagggcggaggtattggcgcgcctcaatccgaaggcgtggctgatagattggcgcggcagccatgttcttggattgagccgcgtcaatatctccccttgcctgtcccgtacctagctagcttgcttgcctcactgatcgatgtcgtccctatttcatggagaagctgatgattgattattctcacaagcaagaactgtctgatctgttgcctgcatcgatcaggatctatatgctggagagttcacaagaacatggacagaactcgcttcaacaaccgatcaatcgattgattaggtatgtacctacctcatatgcctcagctcttcgttatggatttcttcaaccgaagggtcagtaagctcttggttccatgccactgcgtgaactaagcgttcacaaaatccgttccmcggcatgaaccaagcactcaaaatcgcatgcagcatctttcgtttcaaaaaaaaattgacttytgaaaacaatagatgaatcagtttcaaacatatatgattatccattttctcaaccgggaatttatatctcgttgggatgcaaaaccgttcagtagtaaaactactccacgagtataaactgtttcagttattttactattaattagttacccgtatgctgttatggtttctatatatctataagtaaaccttacttaaataagatagttatacaaaaaaaaaaaaaaaa

SEQ ID NO: 248 - DNA, 660 bp, Arabidopsis thaliana
caagaaaaaacattgaaatagctcatgttgtctctttctcattttcatatctgctaaaaaaagaaccgtgttttctaaactggtttaacggtaagtacctgtctctagtaacttacctatcaatttgttccaatcatttacttgctttgacttatttggtttccttttgttttgtttttctttaatatgtggatggagtttggtgtaataagcaactgaagagtcgatgagcgcactatcggacatcaaatacgagatattggtgcggttcaatcagaaaaccgtactcttttgttttaaagatcggtttatttgattgagccgtgccaatatcacgcgtttaaatagtttaaagattctatgttagttgatgtgatcaatcaaggtatgaatctatatcaattctcttatgcatagttttatatttacagagatgaggtattatcaatgtctatcgtcgaggatcacgctcttacttatgttatatttctatataattttattaattagttttctaaaagagaaggacaatttaaaattattttaaagagttttttttaagtagttttgttttcatgtttatcttctgcaggctctgaagttaggatagtaacaagaaaaaagacagaaaaaaagaagaaaattcatatacattcgtga

SEQ ID NO: 249 - DNA, 225 bp, Medicago truncatula
gaataagtgaatattatcgatatttatatcatatatcaacttttcttctgtgcttgcttgcaaatttgcaattaagcttttttgatcttatgtaagagaatattattgatgatggtgtttgggaagccgaaaaaagcgatgttggtgaggttcaatccgaagacggatttacatgtatagagttgtaaaatacgatctcagattgagccgcgccaatatcacttt

SEQ ID NO: 250 - DNA, 367 bp, Medicago truncatula
ccacaaaactataactagctagaagctttaatcgccttatttattataataataataataaatatggcttcagctgcaaaagtatacatggcgtgatattgatccggctcatctatatcttcaagttcaatcatccatattcatatcaatttcagacgagccgaatcaatatcactcttgtttgcttcattgcatattaattatatacttcatttataagttatagtttgccatatatatattagattgattctgcagaagtagacaggagtggtgttgtttctgctcatcttattaaataatgaatgaatgaatgacatttgcttacttataagacgagccgaatcaatatcactccagtacacct

SEQ ID NO: 251 - DNA, 712 bp, Arabidopsis thaliana
ctctctctctctctctctctcatctgtgttctagatctcaccaggtctttctctggttaatatatggcttccaagatctggtaatatgttataaatacgtcatacttaagcttttttcaaatcaaaaatagaaatttgtgggtttgtctcgttttactattttagcagtatatattaagaagttcagatgttattcgatcatctgtttttgcttcccctctgccatctttatcttttagggtttcaattctttttcacttttttcttctggtttggagatggttaggttccaactaagtatacgagattaaatttgacatcttagttacttcaaaattccttcaatcaaaacaagtcatctcgactattccgccatgtttgtatatacatatttatatattatatatatgaaggtacgagtttctagtgtctataaattaagaaggttaagtaccatatagatgatatttgttaagtagtaagtcactcaaagtttgagtttgggtttgagtttgagtttgagtttgagtttgagagacaaaagattactacaagaagattgttaaacaaaaatggaagactaatttccggagccacggtcgttgttggctgctgtggcatcatcaagattcacatctgttgatggacggtggtgattcactctccacaaagttctctatgaaaatgagaatcttgatgatgctgcatcggc

SEQ ID NO: 252 - DNA, 714 bp, Arabidopsis thaliana
acttgcacctctcactccctttctctaactagtcttgtgtgcacccatttatgtgtacgtactattatctcataaataaatatttttaaaattagatgcatttattgatatgaaaaagttacaagattagtttgttgtgtgtgagactttggatcgacagatcgaaaaattaactaaccggtcagtattgaatatcaactattatatgctccatgcattcgcttatagtttcacacaatttgttttcttcacggtctaaaatcagaagattccatatattttcttatgacgtaaaaggaccacttataagttgacacgtcagcccttggattcgtgaggtttttctctctacttcacctatctacttttcctcatatcccactgcttttctccttcttgttcttgtttttctcgtttttttcttcttcttctccaagaaaatagagatcgaaaagattagatctattttgtgtagcaagaaattatcattttcgtttcttcattcatatattgttctattatgttgtacaataatagatactcgatctcttgtgcgtgcgtaaattttatacaagttgtcggcggatccatggaagaaagctcatctgtcgttgtttgtaggcgcagcaccattaagattcacatggaaattgataaataccctaaattagggttttgatatgtatatgagaatcttgatgatgctgcatcaac

SEQ ID NO: 253 - DNA, 324 bp, Arabidopsis thaliana
tcaccaaataggctcttctttatcgcttcatatatataaaagtctacatctatctctttctaggtcactagctagactctagattaaggattgaaattagggtttcatgtttccagcaaaatggtgccgtcttgagtcttgaaaagatccaagacaaaaccaaatcactacatacatccctatcatcaaccagctactgttcgctgttggagcatcatcaagattcacaaatcatcaagtattcgtgtaaataaacccatttatgattagatttttgatgtatgtatgagaatcttgatgatgctgcagctgcaatcagtggct

SEQ ID NO: 254 - DNA, 531 bp, Arabidopsis thaliana
tgtcatattgagaactctttagcctttggcttctgttcctgacacttgtatagtgaagtgggcttgtgttatatagatgggatctctctctttatttaaaagtcaattagagatcttgatgctacttctgtccctttccaagtgattttacgtcgaccaactagcttttttcatatgagtgtatatattcatgtacctatctctctcaattgcttctcaccaaaatcatcttgctgattcatttgctgtctgaatcctcttgctttcctctttgctttttcatttgttgatttaaaccatgggagttcccaactttagacctcgaaaccgataaggatctttctctgcggttgaaatagctaggttctcgatgaataggctagcctttggtggatgttatcagccagtagtcgcagatgcagcaccattaagattcacaagagatgtggttccctttgctttcgcctctcgatccgcagaaaagggttccttatcgagtgggaatcttgatgatgctgcatcagcaaatac

SEQ ID NO: 255 - DNA, 618 bp, Arabidopsis cebennensis
ttgtatccatagtgtatttcctcgcatctaccatccattttctacgcctctctctctctctttctccatcaaatcttgttttgttcaaactctctctctcatcaattctctccatacaatacatgcatacatacatacataccatctctaatatttcatcaatcttcttttgttccaaacgctctttctctccatttacatacatacgaatcattgttgtcatagatccgtttagaattgctttaacttttagatgagatctagggtttctttctttttcttcaaaatcatgctttttcgcttgctaggttatagatccatgtaagtttagagtagatgtacacacacacgctcggacacttattaaatacatgttgatacacttaatactcgctgttttgaattgatgttgtaggaatatataaatgtagagagagcttccttgagtccattcacaggtcggatatgatccaattagcttccgactcattcatccaaataccgagtcgccaaaattcaaattagactcgttaaatgaatgaatgatgcggtagacaaattggatcattgattctctttgattggactgaagggagctccctctctcttctgtattcc

SEQ ID NO: 256 - DNA, 660 bp, Arabidopsis halleri
ttgtatccatagtgtatttcctcgcatctaccatccattttctacgcctcactctctctttctccatcaaatcttgttttgatcaaactctctctctctctctctcatcaattgtctccatacaatacatacataccatcatctttcccatctctaatatttcatcaatcttcttttgttcaaacgctcttcctctccatatacatatacatacatacgaatcacattggtgtcatagatccgtttagaattgctttaacttttagatgagatctagggtttctttgtttctttcgttttcttcaaattttgctgcatattctccaagatcatgatttttcgcttgctaggttatagatccatgcaaatatagagtagatttacacacacacacgctcggacacttattacatacatgttgatacacttaatactcgctgtttttaattgatgttgtaggaatatatatatgtagagagagcttccttgagtccattcacaggtcgtgatatgatccaattagcttccgactcattcatccaaataccgagtcgccaaaattcgaactagactcgttaaatgaatgaatgatgcggtagacaaattggatcattgattctctttgattggactgaagggagctccctctctcttctgtat

SEQ ID NO: 257 - DNA, 632 bp, Arabidospis lyrata
ttgtatccatagtgtatttcctcgcatctaccatccattttctacgcctctctctttctccatcaaatcttgttttgttccaactctctctctcatcaattcattccatacaatacatgcatacatacataccatcatcatcttttcccatctctaatatttcatcagtcttcttttgttacaaacgctctttctcgccatatacatacataagaatcattgttgtcatagatccgtttagaattgctttaacttttagatgagatctagggtttctttctttttcttcaatttttgctgcatattcttcaaaatcatgatttttcgcttgctaggttatagatccatgcaaatatagagtagatgtacacacattcacgctcggacacttattacatacatgttgatacacttaatactcgctgttttgaatggatgttgtaggaatatatatgtagagagagcttccttgagtccattcacaggtcgtgatatgatccaattagcttccgactcattcatccaaataccgagtcgccaaaattcgaactagactcgttaaatgaatgaatgatgcggtagacaaattggatcattgattctctttgattggactgaagggagctccctct

SEQ ID NO: 258 - DNA, 646 bp, Arabidopsis thaliana
ttgtatccgcagtgtatttcctcgcatctaccatcccttttctacgcctctctccctctctctctttctccatcaaatcttgttttgttcaaactctctctctctcatctattctctccatacaatacatgaatatacatacataccatcatcttcttttcccatctctagtttttcatcaatcttctgatgttccaaacgctctatctcttcatatacatacatacgaatatattattgttgtcatagatccatttagaatcactttagcttttagatgagatctagggtttctttgttttctttcaaattttgttgcatattcttctaaatcatggtttttcgcttgctaggttatagatccatgcaaatatggagtagatgtacaaacacacgctcggacgcatattacacatgttcatacacttaatactcgctgttttgaattgatgttttaggaatatatatgtagagagagcttccttgagtccattcacaggtcgtgatatgattcaattagcttccgactcattcatccaaataccgagtcgccaaaattcaaactagactcgttaaatgaatgaatgatgcggtagacaaattggatcattgattctctttgattggactgaagggagctccctct

SEQ ID NO: 259 - DNA, 660 bp, Brassica rapa
ttgtatccattgtgtatttccttgcatccatcaataaattttatgttacgcctctctattatttctctctacatcacactgtcttatgtttaagctctacttctcagcaattctctccacccaatacatgcatacataccatcatcgtatcgctctaatttttctatcaatcttgtatccttccacaaattatcttatgtctcccattttaaatcctacatagatccacacatacgaattattcttgtctgaagatccatccatttacgattgctttaacttttacatgagatctagggcttctttatttttcttcaaatcttgctgcatatatttcaagatcatgcttttcggcttgctagggttctagatccatggatgtatagcgtacatacatacacgcactaattcatacctgtagtttgtacggagaacatcataaaatatcactgtttggaattaatcgtgtaggaaatatagataggtagggagcttcctttagtccattcacagatcatgatatgatccaattagcttccgactcattcatccaaataccgagtcacgaaaatttcaacttagactcgttaaatgaatgaatgatgcggtaaacaaattggatcattgattctctctgattggactgaagggagctccctc

SEQ ID NO: 260 - DNA, 932 bp, Carica papaya
ctatatccctgtcaaatagtacttggttttgttttagccacaaatcttctggtcttgcaaagttccttctgatctctccccctttctcattttttcctcctcttatatatggatcatcaatttgctgtacacacacacacatttactgtagtgataattagctagctaatttgttagtatgtaaattagatcccaagtaccctgttatatttttttaggcttatcctatgcatacctgatagtacaagaacttagtttgtaattaggtacttggtagtagggttagattaattactgtcttgaaagagaacttatccaacaaatagagctatgaagattaaattaggttttagtcttattaagattattatattactagacaaaaacagttaaatttttttaattgggtaattaggtacttagcaatagggttagattaattactgttttgaaagagaacctacctacaaatagagttgaaatgattatgttttagtcttactaagattgtcatatttctggaaaaaaacaaatcttgaaacagataattcagatagtcatgatcaatggaaaaaacatcatgggtgtgtgcttaattaagctaatatatatatatatgaagatataatgttatgcacactagctatgaatttgtaagaataatgaaggataaagatgatatatttagatgttataagtgtaagtaaggtggaatgggttgatgggtagtagtagtagtagtagagatgattggtggagagagcttccttcagcccactcatggatgggtatgaaggggtagaagtagctgccgactcattcattcagccactcagtatgtaaactcgtcccactgttgactgtatgaatgatgcgggagatatttttacatccatctttctctgtgcttggactgaagggagctccttctt

SEQ ID NO: 261 - DNA, 702 bp, Capsella rubella
ttgtatccatagtgtatttcctcgcatctaccatctactattttctacgcctctctctctttatccctctatctctttcttcatcaaatcttcttttgttcaaagtctctctcatcatttttctctatacacatacatgcatccacatacatacatacatataccatcatcttcttttctcatctctagtttttgtttataaattttgttccaaggatctgtatctctccaataaagatacatacaaattattgttgtcatagatctattagaattgctttaacttttatatgagatctaggatttcttccttttctttcaaaatttgctgcatatttttcaaaatcatgatttatcgcttgctaggttctagatccatgcaaatttagagtatttttacacacacacacgcttggacacaagtacatacatgtagttttcttttatgtggtgaaaagtacataacatgtagtttatagttactagtcgctatataatttaaaattgatgttataggaatatatgtacggagagagcttccttgagtccattcacaggtcgtgatatgatccaattagcttccgactcattcatccaaataccgagtctcaccaaaattggaacaagacttgttaaatgaatgaatgatgcggtagacaaattggatcattgattctctttgattggactgaagggagctcc

SEQ ID NO: 262 - DNA, 767 bp, Eucalyptus grandis
tcgtttcccatccccatttcatagaataatgccaccaaacaaagaagcattagctcaaagactaattaccatctgttttattgatagatacgtgcgaaacggtgattgttttttcccaaataagaaaccaaaatgaagcatattcaaaggtggagatatggggagacttccggaaggcaaggggattggaaaaggctcgagatcaaagtgcatagcaacccttcgctaaaggtgaaaaagaatacgaataacttcagtagctcactttaaattccgaaacattaaacaaatcaaatctccctcgccctccttgcctcctctctttacctatataaagccaccgccccttcaatgaaatccacgagtggaaggtcacagtatagtagggtcctgcaaagggagagcgagagcggctccactgtctacctataagcagttcctttcttttgtttacatgtctgttgcacctcaccgagtttttctattctctttcctctggttggttagcagatttctcaggggacttccctcctcccttgaggatccttctcttgaagcgatatgtctcgaatgggtaagagagagagaggaagggagctttcttcagtccacccatgggacgtgttgggttttaattagctgccgactcattcatccaaataccgagcgagagcaagtaacagagctccgtaaatgaatggatgatgcgggagtcttgttgattcccaagctttccgtgattggactgaagggagctccctctatct

SEQ ID NO: 263 - DNA, 612 bp, Gossypium raimondii
gcgtatccttccacttacggattcaccatagctgctatagcccgagtttgcttgtcataatagaaataaactaagggagaaaaaagctctccactctcgcctttttcttcttcgagtctctctctttgactggcctttgtgcaaagatcttccttttttaaacagtcgctttctttactctccctttcccttctttctcttaattgctaaagcagcttccacttccactcactttaacccatgatccatttcaacctgtcacagtggagagcaatttgtatggctaatttccatctcacctattcttttctgtttggggttctctagtctagggttgcatgacatgagagacatggctcttttttttttttttcagttcacaggtgtttatatatgttgttgtgttattttgtcttaaagctttgtgattgatgatctgataggtaagagagagctttcttcagtccactcatgggatggggatggggtttaattagctgccgactcattcatccaaatactgtgttacaaaacccagtaaatgagtgaatgatgcgggagacaaattgaatcctaatcttcctgtgcttggactgaagggagctccctccc

SEQ ID NO: 264 - DNA, 675 bp, Medicago truncatula
atttatccaatcatgttgctctcacttcttttcagcagttctgttgatatcacccttttagttgaagctttggattcatgactttatgagatggtaaatctttaaattaagtttaagtatgcacttgatttgtttatataatttgtttatttagattttaaaccctaagttgacttttttaatttgatttaaattatgatatgattgttatttggcttaccatggtcataatttagggtttagaagatgcatgtatatcttgaattgtttatggtaataaaggggttaggatttctccttttggtgaagtgagaaaatctcataattttgttctgaaggtagtttttaagatttagggttatgggttctttgtttgaatgctttttcaagtctttttcaatgatatttgcctagatctgttttaattttgaattaaaattctgggtttggattaatattattgaagattattattaattaatttattagaaatagatgaagagagcttccttcagtccactcatggaagggtaaggggtttgaatttacctgctgactcattgattcaaacacaatagacaattatggggttatgctattgtgaattgtgtgaatgatgcaggaggtgaatttcttccttttcttctttgcttggactgaagggagtctcccttt

SEQ ID NO: 265 - DNA, 866 bp, Oryza sativa
ttatatctgacgcgttgtaatcctgtttaattagggctttgcccatttcttttgaccccttccggacattcgctagttggaaccttgttttactcctagcagtgtactgtgtagtacttattacgagcaaacgtaaaaataaataaatggaaatgatacaaaggccgtgtttaattttaaaattttttttcaaactttcaacactttacatcccataaaaagcttactatacatacaaacttccaaccttttcgtcacatcgtatctaatttcaactaaacttttaattttagcgtgaactaaacacagccgaagcccggccacattctcactatttttattcattttatcatgcctgtgatgtcacgccttggccctatttaataggccttctccatttctctccatatgatgtcttctcttctctatccctcttgccatcttctatcttccctcttgcacccatctttgtgataacttctactagctcctctcctactaccagtcataccactctcacaaatcctccaagatccgcatggggagaagctccaaaagtttcgtggttagtttaatttcatgcttgtttgctgccgtttttcatgttgatctgatcttaatatatgtagactgctgttaacatattcttttaatttgatggaagaagcgatcgatggatggaagagagcgatccttcagtccactcatgggcggtgctagggtcgaattagctgccgactcattcacccacaatgccaagcaagaaacgcttgagatagcgaagcttagcagatgagtgaatgaagcgggagagtaacgttccgatctcgcgccgtctttgcttggactgaagggtgctccctcct

SEQ ID NO: 266 - DNA, 801 bp, Physcomitrella patens
tgggatccacacgagtaattattccctctctcatgcatcacaacttggacttgcccagcttttacctctctccatgttccaccgtcggagatcctcggtgctgctacccccgttcggccaaacccaacccaaccctaggtgtctgccggacctccgcttcccctcctgcttcaccccctgcaccgcttaaatttgcacctcgtagtatttatctatgccccatttcagatgacttgcatgacacccatctggattcgtctccaggcgccttgtcgtatctattcgctatcagtctttctttcagtctgtctttctgccaagcacaccgtgctggtggtggtgctatcagtcgaagcagtcgccgaagggtccttgtatccagccctcaccggagacagttcgcttcggggtggggagaactgttgagaccgtcgatgttgcatgcagcagcactggcgaaggtgcttctgatactgggtattccagcctcgccgctcggtgcactgcaggtacgtggttacatgacactactgtgtgggtagtctgggcacaagtagatcgacatgccagatttggcccgtatgcgtgtatgtgcggttatgttcccgtttcgattgcggataccttgattgtggagctccgtttcggtccaatagtggctgcgacggaaggtggtcccgctgccgaatcacacgtccgggttgcttatcggggcagggccccgatacggtatccgaacgtttgtcccgggaactggtcgaccttccgcccggcgtctcttggactgaagggagctccact

SEQ ID NO: 267 - DNA, 819 bp, Thellungiella halophila
ttttatacaaataatgttcgataacactaaaccctagccatccaactaatagacaaaaccctacttgtaatttacaaccgcaaattcccagagaacagagtaactacgagagagagatggagattcaaattaaaaagaaaaacttatatataatgaatacacaaaagctacctaatctgtatatatatatatataaatatgtcttcattaaattaatggtcgtggaatagaaaaaggaaaacctaatttgatcgctagggcttatcagagtaaagatggttaaccttcaaaagatgactaattaaccggggagataattaaaagattaaatacgccaacagagagttaagagataccagatttaaattccacaatttggtcatgttcttcttcacgtattcatgacgatgtctgaattatagagaaacccaaaatataaaatgttaattttaccagacatttacataccaataactctatgacgatatgtaaagtaagcaaggcatgtttttatgcagggaagattgaaaattcaagattaatcaagaaaattggaataccaaaaagagagggagctcccttcagtccaatcagagagaatcaatgacccaatttgtctaccgcatcattcattcatttaacaagtctagctcgaattcttggtgactcggtatttggatgaatgagtcggaagctaattggatcatatcacgacctatgaatggactcaaggaagctctctacaaatgtattcctaccacatcaacccaaatatagtgattacagatgctgttctcactgtagactacatttacgttt

SEQ ID NO: 268 - DNA, 503 bp, Arabidopsis thaliana
agacatctcttcttctctcatctctcttttcttctctcttttcctcacataaactctctttttttactattaaatccatatggtacctcaaattaatctatggtcatctagggttatcttgaagattagaattgattctagcacgcacagagaggaagatcattgcatccagaatcacaaacatggcctatcttttatcttttctttttgatctaagtcactgttttatgctatatatagtataatcaaattctttacatgtgcttgtatgtatgcgtatatatagtaacggaattgttaatatgcttatagatgttgagttggtggaggaagagagctttcttcggtccactcatggagtaatatgtgagatttaattgactctcgactcattcatccaaataccaaatgaaagaatttgttctcatatggtaaatgaatgaatgatgcgagagacaaattgagtcttcacttctctatgcttggactgaagggagctccct

SEQ ID NO: 269 - DNA, 365 bp, Arabidopsis thaliana
tcttattccatcacaatcatctagggttttaagccaagcttatatagcccgtcataaagagaactcatctgcctctctctcaataccaataaatatcaccaccgtccttctctcctatcactattcaatctatcgcaaactcctttatgtctctccaattttatgagagggtttccttcaagaacacagtaaaatagattggatctttaaacttttgttccttttcatgagggtttgacaaagattttcttacagtcatctttggcattctgtccacctccttctatacatatatgcatgtgtatatatatatgcgtttcgtgtgaaagaaggaggtgggtatactgccaatagagatctgttag

SEQ ID NO: 270 - DNA, 134 bp, Arabidopsis thaliana
ttgtatcatgacagagcaagaagaagaaagtcaaatgtccacatgagttccctttaacgcttcattgttgaatactcaaagccacattggtttgtatataacactgaagtgtttggggggactcttggtgtcat

SEQ ID NO: 271 - DNA, 229 bp, Arabidopsis thaliana
tttcaaaccctaacactcttataaaccgattcgccaaaatgtatctacaatatattgataatgtaatatctatatattcaaacaatcgtcgtgttggtcggatgttttctagagttcctctgagcacttcattggagatacaattttttataaaatagttttctactgaagtgtttgggggaactcccgggctgattcggtattttaaattcagtagactagctagctg

SEQ ID NO: 272 - DNA, 220 bp, Arabidopsis thaliana
tggtaatagaaatgagcaaggagatatttttttcccctgggtttgaatgaacatcattgagtgcatcgttgatgtaattttacttattttattccattgttgaattaattaaagaagtatatatcagcgttgcattcaattatgtttttctaattttcaggaaatacaaaaaaaatgaaaaaaaaaaatcacttaaaagaccttgagagttcttttgact

SEQ ID NO: 273 - DNA, 225 bp, Arabidopsis thaliana
ggatatcgaaactcaaactgtaacagtccttttattactggtttagaagatagataaatattgttaaggtagtggatctcgacagggttgatatgagaacacacgagcaatcaacggctataacgacgctacgtcattgttacagctctcgtttcatgtgttctcaggtcacccctgctgagctctttctctaccgtccatgttttatcaacgccgtggcccgtg

SEQ ID NO: 274 - DNA, 165 bp, Arabidopsis thaliana
tcttatagagatgaagagaaacatgtaaactcactagttttagggcgcctctccattggcaggtcctttacttccaaatatacacatacatatatgaatatcgaaaatttccgatgatcgatttataaatgacctgccaaaggagagttgccctgaaactggttc

SEQ ID NO: 275 - DNA, 187 bp, Arabidopsis thaliana
caataactcaaaatgcaatgtgaaatatgaagaatatattaaatagtagtgaagatgcatgtttatgaagacagagagataatgtatggttggattactgggcgaatactcctatggcagatcgcattggctagatatgcaagtaaaatgcttctctgccaaaggagatttgccccgcaattcatcc

SEQ ID NO: 276 - DNA, 235 bp, Arabidopsis thaliana
atttaggtctctcttcttcttcttctttttcttcttgagcgccggcgaaaaaagtctctgtgagaaaaagatacgacgattgtcattagaagagtcgtattacatgttttgtgcttgaatctaattcaacaggctttatgtaagagattctttaacaattcctataatctttgttgttggattagattcacgcacaaactcgtaatctgtcttttcgatttttaccagatctgtc

SEQ ID NO: 277 - DNA, 944 bp, Arabidopsis thaliana
aattatatccatggtcatggctcatcattagtcgcactgctctccttttctcaaagtttaaattcgacatttggtaaaatgatgaaacctcgatggaactgctctctttatggaatcacggaatggacaaataatcaaaatcagaaatcgaagcgaaaagggaggagaaaaacgcagatttggaggattggggacagattagatactgttgaatgcatcactctaatgctatcagcctattaatagcgtcctatattttcgaagacttttaatgtttagggttatggatttttcgagcgaagcatggagagatgttgaattggatactataggatttggtacaacacatacatatgttctgcttctgcaaaactaacatatcaagttcagagaaaccagtaagtcgttgaatattttattatccattcaacgctttcttcttttggatcatgtcttgtttgcttgaccacttcttcttgcttaagaggatggacaatatataaaaactggagccttctttttctatgaatgcttatcatcgcggagttgatctgttcaattcacctgccattggatgctttttttatatatacttcactgttcaatttcagatgctttagaaggtttgcggagtagctagagaatctggtatcttcagttcttcaatttcagctacttggtatcagcttcgtcattgtatatcaacacattcttaatatataatactactttttcatccattaaaccccttacaatgtcgagtaaacgaagcatctgtcccctggtattgtcttcgagcttggtgtttttttctagccaactccaagttctcgagttgatcattgtttgtattcttgagacattatttggggacgagatgttttgttgactcgatataagaaggggctttatggaagaaattgtagtattatatatcgagagtg

SEQ ID NO: 278 - DNA, 420 bp, Arabidopsis thaliana
ctataaatgctgcttatcatcgtggagttggttctgtaaacatttgaaaattctgaacagtttcacctgccattggatgctttgtttcaatttcaggtgcgttagaaggtttgcagagtagctagagaatctcgtatcttcactttctgctacttggtatcagcttcgtcactttatatcaacacattcttaatatacaatactactttttcatccattaatccccttacaatgtcgagtaaacgaagcatctgtcccctggtattgtcttcgagcttggtgtgtttttctagccagccccaagttctcgagttgatcattgtttgtattctgacacattatttggggacgagatgttttgttgactcgatataagaaggggctttatggaagaaattgtagtattatatattgagaatg

SEQ ID NO: 279 - DNA, 383 bp, Arabidopsis thaliana
tagtataaccgctgatgtacacctaccagcttgataactctttttcgtggtttctgtgtactcgtttctgtttgtacagatacttcttgttcaatttcagatgctttagaaggttttcggagtggctagagatctgttatctgtatgaacagctacttggtatcagcttcgtcattttatcaacacattcttaatatacaatacttctttttcatgcattaagccccttacaatgtcgagtaaacaaagcatgtgtccgctaatattgtcttcgagcttggtatttttgtattctgatacggtatttggggacgacatcttttgttgactcgatataagaagggggtttgtggaagaaattgtagtattatatatcaagaatg

SEQ ID NO: 280 - DNA, 2164 bp, Drosophila melanogaster
tttgtggaacacattcgacccactgaaaaattgatataatttaatgaaagtgcataaaaatggtggacagtgcattaaactgagcattgaacacaaaggccgctcagcaaattgctaattaaaattcacgattgccatttcacctgacacgttgacgattttcattacaattcgattatgtttcgttgcagggaattttaaatgttaattgccaagaatgtttcaacaaattcatttctcattaatgtgtcttttcatttaattttatgttgtatgagctgcacgagaaatgagttgtacttttagttcgacggcagagtcatgaatgttcggcaaagaatgtaataataactatcctctttagacaaatatagatacaaatctatcagattctaaaagtagaataatcaattaatcagaaagctaaaaataaataggcatatttatattttaatgcggatttttgaagttcaacgggagaaatgaatcctttttaccagccacaggcgcaatttgcaacagaaagtgtagcagaagtactcctcgaatatttccctgctccaggagtcatccatgtggtttcgaggcacacatttgacaaactcatgccccgctatttgttgtaaaaacacaatcgcacacatggccgcatttcggcgacttccagagagcggtacacttaaggcggcctgggaaacgcctgcaatctgctggtcgcgaactgcagattgcatccatgtgccaggcgaccatgcgaccatgtgaccatgtgcccgcccgacgcctcgcagcccacatcctgcccatcgagggcacaactcagcgtgggtattgccgctccggctgcttcaagtaggtaaaaaccgagaagattgaggatgaatgtatgagtatgagaaaatactcggcggaacatatgctgccgggcttgacctgaccctgcctcatgtgtgggtctccgatttaattttaggcacctatataaacgcgtgtttacactgcagccagaacacagtcgccgtcttcagttcgcgccgtcaactcctcgatcgatcgatcgcatcgtctcggatcgaatagagctgggcttctgctccggagctacatcgccgtacttgtcggacgagtgtggtgatgaaaagtcgcttagtccgggattcctgccagatctctaagggatgagctggcatcccaggctggccatgtggcgcgaagtatgcgcacaaaaaagtcaaacaaaaaggcgcaattttattacgggcaaccaacgacgaaacaaaacaaaagccaaccgaaaagcagaaacaaagcagcaaaaagtttatgaattttttgtgcaggcgcgtgaaagatgcaaaacgagaaaaaaacatgaaaaaaaaacattaaaaaaaacaaaaaaaatccaaaacagataccgagctgtatccgaaaacgagtggggaaaggggtttcccagtcacatataaacacacttcagtgcgcttaaaaattgctttattgcagttggactataaaaacgcacggcagcgaacaccgcacaacaaaaaggacgagcagaagtgggcaaataaaacgaaagctcttaaacgaaaaacaggaaaatttgcatgccacaaaaataagcataaggatttgccgcgcacaaagtagaagcaaaaaggaattgcccaaatgcagccacaaaagactgtggcaaatgttttgcagcttgcccctttttccctgcaattaccgtcagtcgttgtcattattcagcagattatatggttttgcttattccggaccaccatcatcatcatcattatcatcatcttcggtaagttagacaatcccataaaaaactgtccaagtgagtagtgccaccaaaagttagccgcgttgtggaaaatccaaaacaaagaccatcccatattcagcctttgagagttccatgcttccttgcattcaatagttatattcaagcatatggaatgtaaagaagtatggagcgaaatctggcgagacatcggagttgaaactaaaactgaaatttgattgaaacagaagtagaaccgtaatgaaatgaatgaaatattaacccgtttctacaatccctgaataaaattattaattaattatagagcgggctaattttacaatatatattgatttttttttgaag

SEQ ID NO: 281 - DNA, 919 bp, Drosophila melanogaster
attcttttttggtgctcgatcgtgacggtttgctcgcgctctccgctgcgccgctctttccgttgcatatgtgtgcgggcgttattgtgcatgtttccggtggccgaaaaaaaatagtaaaataaaatatagaaaacagaaaccaagaataataacagccatacgataaacagtgtgccaatgtgtgtgtctgtgtgtgtgtgcatctcgcgtaacaacaataattgcatttatcggatggcgccagcttcaatttaattataaataacatgttcaactttttatactattttccctgcgtcaaagtgggcgttgcaactgcccccggaaaatcacgcgccccggttcaaagttaaagtttgctgggtaacgcacacacacacacacacaatcactcacacgcggtcacacgcacatttcaataaactaatggagcctggctttgtttttgttttatttccaacccacttgagcacacagcacacacagagagaaaaatcaatactcgttatgggattaaatttacaaagcgcaaagcaaagcgacaaacaaaattcaaaagaaagaaaaaaaaacactcaaataaactcacaaagaattccttatcgccaagggggccaatgttctaaggttctttcgccttgagaactttgagcttcctctggcaaaggagattataatgtacaaataatgttgcaataaccagttgaaaccaatggaataccgaatcttgctaattagcaaggacatctgttcacatcttaccgggcagcattagatcctttttataactctaatactgtcaggtaaagatgtcgtccgtgtccttaaccttcagtaccaccaacagcagcagcagcaccaaaaaaaaaaaaaaaaaaatgcgtaaaaatccaaacaaatcataaaagtcgaagga

SEQ ID NO: 282 - RNA, 20 nt, Arabidopsis thaliana
ugacagaagagagugagcac

SEQ ID NO: 283 - RNA, 20 nt, Arabidopsis thaliana
ugacagaagagagugagcac

SEQ ID NO: 284 - RNA, 20 nt, Arabidopsis thaliana
ugacagaagagagugagcac

SEQ ID NO: 285 - RNA, 20 nt, Arabidopsis thaliana
ugacagaagagagugagcac

SEQ ID NO: 286 - RNA, 21 nt, Arabidopsis lyrata
uuuggauugaagggagcucua

SEQ ID NO: 287 - RNA, 21 nt, Arabidopsis thaliana
uuuggauugaagggagcucua

SEQ ID NO: 288 - RNA, 21 nt, Capsella rubella
uuuggauugaagggagcucua

SEQ ID NO: 289 - RNA, 21 nt, Arabidopsis thaliana
uuuggauugaagggagcucuu

SEQ ID NO: 290 - RNA, 21 nt, Arabidopsis thaliana
ugccuggcucccuguaugcca

SEQ ID NO: 291 - RNA, 21 nt, Arabidopsis thaliana
ugccuggcucccuguaugcca

SEQ ID NO: 292 - RNA, 21 nt, Arabidopsis thaliana
ucaaugcauugaaagugacua

SEQ ID NO: 293 - RNA, 21 nt, Arabidopsis thaliana
ucgauaaaccucugcauccag

SEQ ID NO: 294 - RNA, 21 nt, Arabidopsis thaliana
ucgauaaaccucugcauccag

SEQ ID NO: 295 - RNA, 24 nt, Arabidopsis thaliana
uugaagaggacuuggaacuucgau

SEQ ID NO: 296 - RNA, 21 nt, Arabidopsis lyrata
uggagaagcagggcacgugca

SEQ ID NO: 297 - RNA, 21 nt, Arabidopsis thaliana
uggagaagcagggcacgugca

SEQ ID NO: 298 - RNA, 21 nt, Brassica rapa
uggagaagcagggcacgugca

SEQ ID NO: 299 - RNA, 21 nt, Carica papaya
uggagaagcagggcacgugca

SEQ ID NO: 300 - RNA, 21 nt, Capsella rubella
uggagaagcagggcacgugca

SEQ ID NO: 301 - RNA, 21 nt, Gossypium raimondii
uggagaagcagggcacgugca

SEQ ID NO: 302 - RNA, 21 nt, Medicago truncatula
uggagaagcagggcacgugca

SEQ ID NO: 303 - RNA, 21 nt, Oryza sativa
uggagaagcaggguacgugca

SEQ ID NO: 304 - RNA, 21 nt, Arabidopsis lyrata
ucggaccaggcuucauccccc

SEQ ID NO: 305 - RNA, 21 nt, Arabidopsis thaliana
ucggaccaggcuucauccccc

SEQ ID NO: 306 - RNA, 21 nt, Brassica carinata
ucggaccaggcuucauccccc

SEQ ID NO: 307 - RNA, 21 nt, Brassica juncea
ucggaccaggcuucauccccc

SEQ ID NO: 308 - RNA, 21 nt, Brassica napus
ucggaccaggcuucauccccc

SEQ ID NO: 309 - RNA, 21 nt, Brassica oleracea
ucggaccaggcuucauccccc

SEQ ID NO: 310 - RNA, 21 nt, Brassica rapa
ucggaccaggcuucauccccc

SEQ ID NO: 311 - RNA, 21 nt, Arabidopsis thaliana
ucggaccaggcuucauucccc

SEQ ID NO: 312 - RNA, 21 nt, Arabidopsis thaliana
ucggaccaggcuucauucccc

SEQ ID NO: 313 - RNA, 21 nt, Arabidopsis thaliana
ugaagcugccagcaugaucua

SEQ ID NO: 314 - RNA, 21 nt, Arabidopsis thaliana
ugaagcugccagcaugaucua

SEQ ID NO: 315 - RNA, 21 nt, Arabidopsis thaliana
cagccaaggaugacuugccgg

SEQ ID NO: 316 - RNA, 21 nt, Arabidopsis thaliana
uagccaaggaugacuugccug

SEQ ID NO: 317 - RNA, 21 nt, Arabidopsis thaliana
ugauugagccgcgccaauauc

SEQ ID NO: 318 - RNA, 21 nt, Arabidopsis thaliana
uugagccgugccaauaucacg

SEQ ID NO: 319 - RNA, 21 nt, Medicago truncatula
ugauugagccgcgucaauauc

SEQ ID NO: 320 - RNA, 21 nt, Zea mays
ggauugagccgcgucaauauc

SEQ ID NO: 321 - RNA, 21 nt, Arabidopsis thaliana
uugagccgugccaauaucacg

SEQ ID NO: 322 - RNA, 21 nt, Medicago truncatula
agauugagccgcgccaauauc

SEQ ID NO: 323 - RNA, 21 nt, Medicago truncatula
cgagccgaaucaauaucacuc

SEQ ID NO: 324 - RNA, 21 nt, Arabidopsis thaliana
agaaucuugaugaugcugcau

SEQ ID NO: 325 - RNA, 20 nt, Arabidopsis thaliana
gcagcaccauuaagauucac

SEQ ID NO: 326 - RNA, 21 nt, Arabidopsis thaliana
agaaucuugaugaugcugcag

SEQ ID NO: 327 - RNA, 21 nt, Arabidopsis thaliana
ggaaucuugaugaugcugcau

SEQ ID NO: 328 - RNA, 21 nt, Arabidopsis cebennensis
uuggacugaagggagcucccu

SEQ ID NO: 329 - RNA, 21 nt, Arabidopsis halleri
uuggacugaagggagcucccu

SEQ ID NO: 330 - RNA, 21 nt, Arabidospis lyrata
uuggacugaagggagcucccu

SEQ ID NO: 331 - RNA, 21 nt, Arabidopsis thaliana
uuggacugaagggagcucccu

SEQ ID NO: 332 - RNA, 21 nt, Brassica rapa
uuggacugaagggagcucccu

SEQ ID NO: 333 - RNA, 21 nt, Carica papaya
uuggacugaagggagcuccuu

SEQ ID NO: 334 - RNA, 19 nt, Capsella rubella
uuggacugaagggagcucc

SEQ ID NO: 335 - RNA, 21 nt, Eucalyptus grandis
uuggacugaagggagcucccu

SEQ ID NO: 336 - RNA, 21 nt, Gossypium raimondii
uuggacugaagggagcucccu

SEQ ID NO: 337 - RNA, 22 nt, Medicago truncatula
uuggacugaagggagucucccu

SEQ ID NO: 338 - RNA, 21 nt, Oryza sativa
uuggacugaagggugcucccu

SEQ ID NO: 339 - RNA, 20 nt, Physcomitrella patens
cuuggacugaagggagcucc

SEQ ID NO: 340 - RNA, 20 nt, Thellungiella halophila
uggacucaaggaagcucucu

SEQ ID NO: 341 - RNA, 21 nt, Arabidopsis thaliana
uuggacugaagggagcucccu

SEQ ID NO: 342 - RNA, 20 nt, Arabidopsis thaliana
uuggcauucuguccaccucc

SEQ ID NO: 343 - RNA, 21 nt, Arabidopsis thaliana
cugaaguguuuggggggacuc

SEQ ID NO: 344 - RNA, 21 nt, Arabidopsis thaliana
cugaaguguuugggggaacuc

SEQ ID NO: 345 - RNA, 21 nt, Arabidopsis thaliana
ucauugagugcaucguugaug

SEQ ID NO: 346 - RNA, 21 nt, Arabidopsis thaliana
uguguucucaggucaccccug

SEQ ID NO: 347 - RNA, 21 nt, Arabidopsis thaliana
ugccaaaggagaguugcccug

SEQ ID NO: 348 - RNA, 21 nt, Arabidopsis thaliana
ugccaaaggagauuugccccg

SEQ ID NO: 349 - RNA, 21 nt, Arabidopsis thaliana
uuagauucacgcacaaacucg

SEQ ID NO: 350 - RNA, 22 nt, Arabidopsis thaliana
uuggggacgagauguuuuguug

SEQ ID NO: 351 - RNA, 22 nt, Arabidopsis thaliana
uuggggacgagauguuuuguug

SEQ ID NO: 352 - RNA, 21 nt, Arabidopsis thaliana
ccccuuacaaugucgaguaaa

SEQ ID NO: 353 - RNA, 22 nt, Drosophila melanogaster
uggaauguaaagaaguauggag

SEQ ID NO: 354 - RNA, 23 nt, Drosophila melanogaster
uaauacugucagguaaagauguc

SEQ ID NO: 355 - protein, 17 aa, Homo sapiens
MEMALMVAQTRKGKSVV

SEQ ID NO: 356 - DNA, 53 bp, Homo sapiens
tggagatggctctaatggtggcacaaaccaggaaggggaaatctgtggtttaa

SEQ ID NO: 357 - DNA, 1500 bp, Homo sapiens
gccgagcccgggcccagcgccgcctgcagcctcgggaagggagcggatagcggagccccgagccgcccgcagagcaagcgcggggaaccaaggagacgctcctggcactgcagataacttgtctgcatttcaagaacaacctaccagagaccttacctgtcaccttggctctcccacccaatggagatggctctaatggtggcacaaaccaggaaggggaaatctgtggtttaaattctttatgcctcatcctctgagtgctgaaggcttgctgtaggctgtatgctgttaatgctaatcgtgataggggtttttgcctccaactgactcctacatattagcattaacagtgtatgatgcctgttactagcattcacatggaacaaattgctgccgtgggaggatgacaaagaagcatgagtcaccctgctggataaacttagacttcaggctttatcatttttcaatctgttaatcataatctggtcactgggatgttcaaccttaaactaagttttgaaagtaaggttatttaaaagatttatcagtagtatcctaaatgcaaacattttcatttaaatgtcaagcccatgtttgtttttatcattaacagaaaatatattcatgtcattcttaattgcaggttttggcttgttcattataatgttcataaacacctttgattcaactgttagaaatgtgggctaaacacaaatttctataatatttttgtagttaaaaattagaaggactactaacctccagttatatcatggattgtctggcaacgttttttaaaagatttagaaactggtactttcccccaggtaacgattttctgttcaggcaacttcagtttaaaattaatacttttatttgactcttaaagggaaactgaaaggctatgaagctgaatttttttaatgaaatatttttaacagttagcagggtaaataacatctgacagctaatgagatattttttccatacaagataaaaagatttaatcaaaaaatttcatatttgaaatgaagtcccaaatctaggttcaagttcaatagcttagccacataatacggttgtgcgagcagagaatctacctttccacttctaagcctgtttcttcctccatatggggataatactttacaaggttgttgtgaggcttagatgagatagagaattattccataagataatcaagtgctacattaatgttatagttagattaatccaagaactagtcaccctactttattagagaagagaaaagctaatgatttgatttgcagaatatttaaggtttggatttctatgcagtttttctaaataaccatcacttacaaatatgtaaccaaacgtaattgttagtatatttaatgtaaacttgttttaacaactcttctcaacattttgtccaggttattcactgtaaccaaataaatctcatgagtctttagttgatttaaaataaaaaaaaaaaaaaaaaaaaaaaaaaaa

SEQ ID NO: 358 - RNA, 23 nt, Homo sapiens
uaauacugucagguaaagauguc

SEQ ID NO: 359 - DNA, 337 bp, Medicago truncatula
ttagggttttcagctcatggtaataaaaatgtcatctaatgtcttgcatgtgggaatgaggtcatatatgcagccaaggatgacttgccggcgagcctctttcgatacttttatgacataattaatcatgtggatagccaaggtactaaactcactttgcactaaaacaaatatttttgctttagtgcaaacttagtttaggcgcttcgcaacggctagtcaaatgtcctagttccaatgtgattggttgtccggcaagtcgtctctggctacgtaaaggcctccttttttcatgctagatttttgatgatttgatatagccacacatattttggaa

SEQ ID NO: 360 - DNA, 121 bp, Medicago truncatula
aagaggcagagagagtaatgcagccaaggatgacttgccgacaacattggcgaatgttcatgtgatttctgcctcattgtgccggcaagttgtccttggctatgttagtctctcatcttct

SEQ ID NO: 361 - DNA, 114 bp, Medicago truncatula
tgaattcccctccgctttttgatgttggcttgtctcaatcaaatcaaagttcttgaaatttgagttctttagtctgattgagtcgtgccaatatcatattaagcgataaaagtc

SEQ ID NO: 362 - DNA, 367 bp, Medicago truncatula; identical to SEQ ID NO: 250

SEQ ID NO: 363 - DNA, 135 bp, Medicago truncatula
aactgcaacttgaggaggcatccaaagggatcgcattgatcctataatatttcaactttagtcactttaattttctctcatataatacttaattgggatcatgccatccctttggatttctcctttagtagctac

SEQ ID NO: 364 - DNA, 119 bp, Medicago truncatula
aggcatccaaagggatcgcattgatcccaaatctaattaagtccctagctacttaattaacaacttaatttccttaatatctcataatatttgggatcatgctatccctttggattcat

SEQ ID NO: 365 - DNA, 93 bp, Medicago truncatula
tgcttttccacagctttcttgaacttctttcgtatcttaaatctgttttcaagattaaaagtcctagaagctcaagaaagctgtgggagaata

SEQ ID NO: 366 - DNA, 95 bp, Medicago truncatula
tattcttccacagctttcttgaactgcatccaaattgagttcctttgcattgccatggccattgttttgcggttcaataaagctgtgggaagata

SEQ ID NO: 367 - RNA, 21 nt, Medicago truncatula
cagccaaggaugacuugccgg

SEQ ID NO: 368 - RNA, 21 nt, Medicago truncatula
cagccaaggaugacuugccga

SEQ ID NO: 369 - RNA, 21 nt, Medicago truncatula
ugauugagucgugccaauauc

SEQ ID NO: 370 - RNA, 20 nt, Medicago truncatula
gagccgaaucaauaucacuc

SEQ ID NO: 371 - RNA, 21 nt, Medicago truncatula
uccaaagggaucgcauugauc

SEQ ID NO: 372 - RNA, 21 nt, Medicago truncatula
uccaaagggaucgcauugauc

SEQ ID NO: 373 - RNA, 21 nt, Medicago truncatula
uuccacagcuuucuugaacuu

SEQ ID NO: 374 - RNA, 21 nt, Medicago truncatula
uuccacagcuuucuugaacug

SEQ ID NO: 375 - protein, 15 aa, Arabidopsis thaliana
MMLHITHRFESDVGC

SEQ ID NO: 376 - protein, 4 aa, Arabidopsis thaliana
MLYV

SEQ ID NO: 377 - protein, 14 aa, Arabidopsis thaliana
MFMRRGLVYNNIYI

SEQ ID NO: 378 - protein, 17 aa, Arabidopsis thaliana
MMKVCDEQDGEAGHVHY

SEQ ID NO: 379 - protein, 28 aa, Arabidopsis thaliana
MKKRITRINLEEQIKKTLDDSRTRLHSP

SEQ ID NO: 380 - protein, 10 aa, Arabidopsis thaliana
MKKIGSIDSF

SEQ ID NO: 381 - protein, 6 aa, Arabidopsis thaliana
MTCRFK

SEQ ID NO: 382 - protein, 11 aa, Arabidopsis thaliana
MKNENLCGSQG

SEQ ID NO: 383 - protein, 45 aa, Arabidopsis thaliana
MKCMMKKRGLTWRKASCLVAKDDLPDLFRLHDSISNSCILDYYTF

SEQ ID NO: 384 - protein, 7 aa, Arabidopsis thaliana
MFPRESL

SEQ ID NO: 385 - protein, 29 aa, Arabidopsis thaliana
MTLSVFFHSFLELQNFFRFFFFSFDISYA

SEQ ID NO: 386 - protein, 23 aa, Arabidopsis thaliana
MSLAKGELPCHCFRLNTVYNRFC

SEQ ID NO: 387 - DNA, 48 bp, Arabidopsis thaliana
atgatgttgcatatcacacataggtttgagagtgatgttggttgttga

SEQ ID NO: 388 - DNA, 15 bp, Arabidopsis thaliana
atgctgtatgtatag

SEQ ID NO: 389 - DNA, 45 bp, Arabidopsis thaliana
atgttcatgcgtagaggtttggtatacaacaatatatacatataa

SEQ ID NO: 390 - DNA, 54 bp, Arabidopsis thaliana
atgatgaaggtgtgtgatgagcaagatggagaagcagggcacgtgcattactag

SEQ ID NO: 391 - DNA, 87 bp, Arabidopsis thaliana
atgaagaagagaatcactcgaattaatttggaagaacaaattaagaaaaccctagatgattctcggaccaggcttcattccccctaa

SEQ ID NO: 392 - DNA, 33 bp, Arabidopsis thaliana
atgaagaagatcggtagtattgattcattttaa

SEQ ID NO: 393 - DNA, 21 bp, Arabidopsis thaliana
atgacttgccgatttaaatga

SEQ ID NO: 394 - DNA, 12 bp, Arabidopsis thaliana
atggtgacatga

SEQ ID NO: 395 - DNA, 36 bp, Arabidopsis thaliana
atgaagaatgagaacttgtgtggtagccaaggatga

SEQ ID NO: 396 - DNA, 138 bp, Arabidopsis thaliana
atgaagtgtatgatgaagaagagaggtctaacatggcggaaagcgtcatgtttagtagccaaggatgacttgcctgatctttttcgcctccacgattcaatttcaaattcatgcattttggattattataccttttaa

SEQ ID NO: 397 - DNA, 24 bp, Arabidopsis thaliana
atgtttccgagagagtccctctga

SEQ ID NO: 398 - DNA, 90 bp, Arabidopsis thaliana
atgaccctctctgtattcttccacagctttcttgaactgcaaaacttcttcagatttttttttttttcttttgatatctcttacgcataa

SEQ ID NO: 399 - DNA, 72 bp, Arabidopsis thaliana
atgtcacttgccaaaggagagttgccctgtcactgcttccgcttaaacacagtctataaccggttctgctaa

SEQ ID NO: 400 - DNA, 331 bp, Arabidopsis thaliana
ctttgtcacttcatacactccctattgtctatatatatatatatacttacacatattcaaacattataatacttaattacacatacatactttatgatgttgcatatcacacataggtttgagagtgatgttggttgttgacagaagatagagagcactaaggatgacatgcaagtacatacatatatatcatcacaccgcatgtggatgataaaatatgtataacaaattcaaagaaagagagggagagaaagagagagaacctgcatctctactcttttgtgctctctatacttctgtcaccacctttatctcttcttctctctaacct

SEQ ID NO: 401 - DNA, 304 bp, Arabidopsis thaliana
atttactcttcaccgccctctctctatatatagtctctatcctcacatattatatatcaaaccgcaagaatgctgtatgtatagtggagggtgatagtgtggttgctgacagaagatagagagcactaaggatgctatgcaaaacagacacagatatgtgtttctaattgtatttcatactttaacctcaaagttgatataaaaaaagaaagaaagatagaagagctagaagactatctgcatctctattcctatgtgctctctatgcttctgtcatcacctttctttctctatttctctctac

SEQ ID NO: 402 - DNA, 245 bp, Arabidopsis thaliana
aaccaaaactcttcaacatttctctctgactacttcatttcctcttcccaacagttaaaaaaagttctgattcgattcaagccaagatccacgtataaagatatgttcatgcgtagaggtttggtatacaacaatatatacatataatagtttgtcgttatgcctggctccctgtatgccacgagtggataccgattttggttttaaaatcggctgccggtggcgtacaaggagtcaagcatgac

SEQ ID NO: 403 - DNA, 240 bp, Arabidopsis thaliana
atacattctctctttctctctctctctctctctcatcccggcccagttatgtggtcggagagaatgatgaaggtgtgtgatgagcaagatggagaagcagggcacgtgcattactagctcatatatacactctcaccacaaatgcgtgtatatatgcggaattttgtgatatagatgtgtgtgtgtgttgagtgtgatgatatggatgagttagttcttcatgtgcccatcttcaccatc

SEQ ID NO: 404 - DNA, 280 bp, Arabidopsis thaliana
tcacacatacctttctttctcttcttcttcttacgaaaagtttcatcacattcacattatctttaactttggtctcttttcttttttgtctcttttctcttcttgataacgtggttctagtcttgattaattcattgttgtgcgatttagtgttgagaggattgttgtctggctcgaggtcatgaagaagagaatcactcgaattaatttggaagaacaaattaagaaaaccctagatgattctcggaccaggcttcattccccctaacctacttatcgc

SEQ ID NO: 405 - DNA, 179 bp, Arabidopsis thaliana
atttagcttcttcttcttcttcttcttctgtctacttacataaagttatccttgctttggtttagggttgagaggaatattgtctggctcgaggtcatgaagaagatcggtagtattgattcattttaaagagtgaaatccctaaatgattctcggaccaggcttcattccccccaacc

SEQ ID NO: 406 - DNA, 376 bp, Arabidopsis thaliana
tagtattcataagcaccaaaacaaatatgtagagatctcctcttccattctctattgttactttcgagaagaaacatacaaaacacatacatttttcttttgtttgtggttttcatatatacaagtgggtatagctagtgaaacgcgaatgtgacgaaagtagtgtgcagccaaggatgacttgccgatttaaatgatctttctttatactctattaagacaatttagtttcaaacttttttttttttttttttttgaaggattcaggaagaaattaggatatattattccgtataaaatacaagatatataaaaccaaaaagaaaaagtaacatgatcggcaagttgtccttggctacacgttactttgtgtcgc

SEQ ID NO: 407 - DNA, 77 bp, Arabidopsis thaliana
actcatcaacaacctcttcataaatacataaatcatataagagaaaatggtgacatgaagaatgagaacttgtgtgg

SEQ ID NO: 408 - DNA, 248 bp, Arabidopsis thaliana
aggcaaaaacatatagagagtaatgaagtgtatgatgaagaagagaggtctaacatggcggaaagcgtcatgtttagtagccaaggatgacttgcctgatctttttcgcctccacgattcaatttcaaattcatgcattttggattattataccttttaaagtataataggtcaaatatcatgttgaatcttgcgggttaggtttcaggcagtctctttggctatcttgacatgctttttccatccat

SEQ ID NO: 409 - DNA, 187 bp, Arabidopsis thaliana
attcactcccttcttcttcttaatctccttacagttacagacattctctcacttgcgttcttgtttcttttacaaaacagatacactatgtttccgagagagtccctctgatattggcctggttcactcagattctcttttactaactcatctgattgagccgtgtcaatatctcagtcctctctcg

SEQ ID NO: 410 - DNA, 246 bp, Arabidopsis thaliana
tctcacaacttcaacttccctctttctctatattacgcttttgcccctcactccctctttccacaattagggtttcgtctgctctacatgaccctctctgtattcttccacagctttcttgaactgcaaaacttcttcagatttttttttttttcttttgatatctcttacgcataaaatagtgattttcttcatatctctgctcgattgatttgcggttcaataaagctgtgggaagatacagac

SEQ ID NO: 411 - DNA, 631 bp, Arabidopsis thaliana
gaataaccaaccagccttctctcaaagcaaaccaaaaagaaaaaccaacattgaaagaggaagttacgataagcggagcagtaatagggcatctttctattggcaggcgacttggctatttgtatcttttgtgttcttgactattggctatgtcacttgccaaaggagagttgccctgtcactgcttccgcttaaacacagtctataaccggttctgctaatatcaatccttcttttggacatgtccaaagccgagattgattgatagagaattggtctctctggctacaaaactagtgcggttctctcgatttaagttttaatagcattcactttgcacattgcatctttcacatcaaatttccatttcatcaaccatctaaacctctttgttagctttgatataagcaacgatctaaagtctaaaaaccattaatcctctgaaaaaaaagacaatttcgatggttctattatgtttctccaatgcagaaattgtatcgtctgaattatagtagattttttctagactaaagtgtaaaccaagacgaatctgcactaacaagacacaccaatagactttacagagaaaggttacgagttttgaaaatattaacggaccatagtcatcgcg

SEQ ID NO: 412 - RNA, 21 nt, Arabidopsis thaliana
uugacagaagauagagagcac

SEQ ID NO: 413 - RNA, 20 nt, Arabidopsis thaliana
ugacagaagauagagagcac

SEQ ID NO: 414 - RNA, 21 nt, Arabidopsis thaliana
ugccuggcucccuguaugcca

SEQ ID NO: 415 - RNA, 21 nt, Arabidopsis thaliana
uggagaagcagggcacgugca

SEQ ID NO: 416 - RNA, 21 nt, Arabidopsis thaliana
ucggaccaggcuucauucccc

SEQ ID NO: 417 - RNA, 21 nt, Arabidopsis thaliana
ucggaccaggcuucauucccc

SEQ ID NO: 418 - RNA, 21 nt, Arabidopsis thaliana
cagccaaggaugacuugccga

SEQ ID NO: 419 - RNA, 21 nt, Arabidopsis thaliana
uagccaaggaugacuugccug

SEQ ID NO: 420 - RNA, 21 nt, Arabidopsis thaliana
uagccaaggaugacuugccug

SEQ ID NO: 421 - RNA, 21 nt, Arabidopsis thaliana
ugauugagccgugucaauauc

SEQ ID NO: 422 - RNA, 21 nt, Arabidopsis thaliana
uuccacagcuuucuugaacug

SEQ ID NO: 423 - RNA, 21 nt, Arabidopsis thaliana
ugccaaaggagaguugcccug

SEQ ID NO: 424 - protein, 13 aa, Medicago truncatula
MVKESFMERLKVR

SEQ ID NO: 425 - DNA, 42 bp, Medicago truncatula
atggtcaaagagtctttcatggagaggttgaaagtgagatga

SEQ ID NO: 426 - DNA, 291 bp, Medicago truncatula
tggataagttaatttatggtcaaagagtctttcatggagaggttgaaagtgagatgaagccaaggatgacttgccggtataatagtaatttgccacaaatctagatagctattagctatgtttggatgggcggtgagattaacaaaattacagcagcattgtgattttgttgatgctttaaagtgtagtttttatcaaaattacagtggttcactgtaattatgagaatctcaccgtcaatctaaatatgcatttagtttcatttccggcaggtcatccttcggctatatt

SEQ ID NO: 427 - RNA, 21 nt, Medicago truncatula
aagccaaggaugacuugccgg

SEQ ID NO: 428 - protein, 20 aa, Artificial Sequence
  Primer
LIVSHLYSEKFDCMRKILRI

SEQ ID NO: 429 - DNA, 20 bp, Artificial Sequence
  Primer
tccccaaattcttgaccaaa

SEQ ID NO: 430 - DNA, 20 bp, Artificial Sequence
  Primer
ttgaggggaaaacatgaacc

SEQ ID NO: 431 - DNA, 20 bp, Artificial Sequence
  Primer
acgaaatccgtctcatttgc

SEQ ID NO: 432 - DNA, 20 bp, Artificial Sequence
  Primer
gggtgaagagctcatgttgg

SEQ ID NO: 433 - DNA, 19 bp, Artificial Sequence
  Primer
tgaggggaatgttgtctgg

SEQ ID NO: 434 - DNA, 19 bp, Artificial Sequence
  Primer
gaagcctggtccgaggata

SEQ ID NO: 435 - DNA, 20 bp, Artificial Sequence
  Primer
cgagtcgccaaaattcaaac

SEQ ID NO: 436 - DNA, 20 bp, Artificial Sequence
  Primer
gctcccttcagtccaatcaa

SEQ ID NO: 437 - DNA, 20 bp, Artificial Sequence
  Primer
gcaactgcagtggaatagca

SEQ ID NO: 438 - DNA, 20 bp, Artificial Sequence
  Primer
gcgaccttcatgggttctaa

SEQ ID NO: 439 - DNA, 20 bp, Artificial Sequence
  Primer
ctcagcatcagcaacgtgat

SEQ ID NO: 440 - DNA, 20 bp, Artificial Sequence
  Primer
aactctgctagggcctcctc

SEQ ID NO: 441 - DNA, 20 bp, Artificial Sequence
  Primer
tcacaactcctcagcattcg

SEQ ID NO: 442 - DNA, 20 bp, Artificial Sequence
  Primer
acccaatcaacagcagttcc

SEQ ID NO: 443 - DNA, 20 bp, Artificial Sequence
  Primer
ggtaacattgtgctcagtgg

SEQ ID NO: 444 - DNA, 20 bp, Artificial Sequence
  Primer
ctcggccttggagatccaca

SEQ ID NO: 445 - DNA, 30 bp, Artificial Sequence
  Primer
tcatcgatgaatatacatacataccatcat

SEQ ID NO: 446 - DNA, 33 bp, Artificial Sequence
  Primer
tccggatcctctaaaagctaaagtgattctaaa

SEQ ID NO: 447 - DNA, 26 bp, Artificial Sequence
  Primer
tcatcgagagagagcttccttgagtc

SEQ ID NO: 448 - DNA, 28 bp, Artificial Sequence
  Primer
tccggatccagagggagctcccttcagt

SEQ ID NO: 449 - DNA, 26 bp, Artificial Sequence
  Primer
tcatcggttgaggggaatgttgtctg

SEQ ID NO: 450 - DNA, 27 bp, Artificial Sequence
  Primer
tccggatccgttgggggggatgaagcc

SEQ ID NO: 451 - DNA, 28 bp, Artificial Sequence
  Primer
tcatcgatgagggttaagctatttcagt

SEQ ID NO: 452 - DNA, 31 bp, Artificial Sequence
  Primer
tccggatcctaatatcctcgatccagacaac

SEQ ID NO: 453 - DNA, 21 bp, Artificial Sequence
  Primer
cgcctcaatttgaatacatgg

SEQ ID NO: 454 - DNA, 20 bp, Artificial Sequence
  Primer
acgcggctcaatcaaactac

SEQ ID NO: 455 - DNA, 23 bp, Artificial Sequence
  Primer
gcactagctggtttcattattcc

SEQ ID NO: 456 - DNA, 21 bp, Artificial Sequence
  Primer
ttgcaaaatttggagagccta

SEQ ID NO: 457 - DNA, 20 bp, Artificial Sequence
  Primer
aagcgatgttggtgaggttc

SEQ ID NO: 458 - DNA, 21 bp, Artificial Sequence
  Primer
cggctcaatctgagatcgtat

SEQ ID NO: 459 - DNA, 20 bp, Artificial Sequence
  Primer
gggcggtgagattaacaaaa

SEQ ID NO: 460 - DNA, 20 bp, Artificial Sequence
  Primer
cctgccggaaatgaaactaa

SEQ ID NO: 461 - DNA, 26 bp, Artificial Sequence
  Primer
tcatcgatgatggtgtttgggaagcc

SEQ ID NO: 462 - DNA, 30 bp, Artificial Sequence
  Primer
tccggatcctacatgtaaatccgtcttcgg

SEQ ID NO: 463 - DNA, 21 bp, Artificial Sequence
  Primer
aggcttcttcataggctctcc

SEQ ID NO: 464 - DNA, 39 bp, Artificial Sequence
  Primer
tcagtccgctcgaggaataagtgaatattatcgatattt

SEQ ID NO: 465 - DNA, 38 bp, Artificial Sequence
  Primer
aaggaaaaaagcggccgcaaagtgatattggcgcggct

SEQ ID NO: 466 - DNA, 67 bp, Artificial Sequence
  Primer
tagcatgttattacaccgcttaagtaagttctgtaagatagagcgcgatattgtttacattagctag

SEQ ID NO: 467 - DNA, 67 bp, Artificial Sequence
  Primer
cgtactagctaatgtaaacaatatcgcgctctatcttacagaacttacttaagcggtgtaataacat

SEQ ID NO: 468 - DNA, 38 bp, Artificial Sequence
  Primer
aaaaggtctcgccataagcatagtggaataatgaaacc

SEQ ID NO: 469 - DNA, 37 bp, Artificial Sequence
  Primer
aaaaggtctcgccatttccatacctgaatttctcctt

SEQ ID NO: 470 - DNA, 38 bp, Artificial Sequence
  Primer
aaaaggtctcgccatcttcatcctcaatatcctaattc

SEQ ID NO: 471 - DNA, 44 bp, Artificial Sequence
  Primer
aggtctcgacacagatatatatactatgtctctttcaattttgc

SEQ ID NO: 472 - DNA, 35 bp, Artificial Sequence
  Primer
aaaggtctcgccatgaccattttcccacgaatatg

SEQ ID NO: 473 - DNA, 36 bp, Artificial Sequence
  Primer
aaggtctcgacacaagcatagtggaataatgaaacc

SEQ ID NO: 474 - DNA, 38 bp, Artificial Sequence
  Primer
aaggtctcgacacagatatatatactatgtctctttca

SEQ ID NO: 475 - DNA, 22 bp, Artificial Sequence
  Primer
gaattcctgcccatggttttcg

SEQ ID NO: 476 - DNA, 22 bp, Artificial Sequence
  Primer
cgaaaaccatgggcaggaattc

SEQ ID NO: 477 - DNA, 23 bp, Artificial Sequence
  Primer
cagtcccgacttaagctcaatac

SEQ ID NO: 478 - DNA, 23 bp, Artificial Sequence
  Primer
gtattgagcttaagtcgggactg

SEQ ID NO: 479 - DNA, 43 bp, Artificial Sequence
  Primer
aaaggtctcctagcttggtcaaacatacatacagtagcactag

SEQ ID NO: 480 - DNA, 46 bp, Artificial Sequence
  Primer
aaaggtctcgcgtaaaattgtactgattgaatgtaaattggtacac

SEQ ID NO: 481 - DNA, 22 bp, Artificial Sequence
  Primer
tagcatgttttcccctcaatga

SEQ ID NO: 482 - DNA, 22 bp, Artificial Sequence
  Primer
cgtatcattgaggggaaaacat

SEQ ID NO: 483 - DNA, 36 bp, Artificial Sequence
  Primer
aaaggtctcctagcactcataactctccccaaattc

SEQ ID NO: 484 - DNA, 37 bp, Artificial Sequence
  Primer
aaaggtctcgcgtagaaagaatgttcgaaaaacaatg

SEQ ID NO: 485 - DNA, 35 bp, Artificial Sequence
  Primer
aggtctccaaatcatgaagcaggcagtaataacct

SEQ ID NO: 486 - DNA, 64 bp, Artificial Sequence
  Primer
aggtctcgcgtactaagcgtaatctggaacatcgtatgggtataatatcctcgatccagacaac

SEQ ID NO: 487 - DNA, 31 bp, Artificial Sequence
  Primer
aggtctcgccatagtggcggagacgaagatg

SEQ ID NO: 488 - DNA, 34 bp, Artificial Sequence
  Primer
aggtctcgccattaatatcctcgatccagacaac

SEQ ID NO: 489 - DNA, 34 bp, Artificial Sequence
  Primer
aggtctccaaattaaactgtcagtgcatggatgt

SEQ ID NO: 490 - DNA, 37 bp, Artificial Sequence
  Primer
aggtctcgacacattcacaaatttttgttgtagagag

SEQ ID NO: 491 - DNA, 37 bp, Artificial Sequence
  Primer
aggtctcgacacattaacaaatttttgttgtagagag

SEQ ID NO: 492 - DNA, 36 bp, Artificial Sequence
  Primer
aggtctcgacactagcagattcacaaatttttgttg

SEQ ID NO: 493 - DNA, 35 bp, Artificial Sequence
  Primer
aggtctcgacaccctcatgataatcgatcttagca

SEQ ID NO: 494 - DNA, 272 bp, Drosophila melanogaster
cgcacacacacacacacacaatcactcacacgcggtcacacgcacatttcaataaactaatggagcctggctttgtttttgttttatttccaacccacttgagcacacagcacacacagagagaaaaatcaatactcgttatgggattaaatttacaaagcgcaaagcaaagcgacaaacaaaattcaaaagaaagaaaaaaaaacactcaaataaactcacaaagaattccttatcgccaagggggccaatgttctaaggttctttcgcct

SEQ ID NO: 495 - DNA, 272 bp, Artificial sequence
  Mutated sequence
cgcacacacacacacacacaatcactcacacgcggtcacacgcacatttcaataaactaagtgagcctggctttgtttttgttttatttccaacccacttaagcacacagcacacacagagagaaaaatcaatactcgttagtggattaaatttacaaagcgcaaagcaaagcgacaaacaaaattcaaaagaaagaaaaaaaaacactcaaataaactcacaaagaattccttatcgccaagggggccaatgttctaaggttctttcgcct